European Patent Application EP 4 714 464 A2, published March 25, 2026. Title: RECOMBINANT HUMAN/BOVINE PARAINFLUENZA VIRUS 3 (B/HPIV3) EXPRESSING A CHIMERIC RSV/BPIV3 F PROTEIN AND USES THEREOF. Applicant: The United States of America, as represented by the Secretary, Department of Health and Human Services. Application EP. The sequence listing filed with the application follows.

SEQUENCE LISTING (153 sequences)

SEQ ID NO: 1 - protein, 574 aa, synthetic construct
  REGION 1..574: note = Recombinant RSV F
MELLILKANAITTILTAVTFCFASGQNITEEFYQSTCSAVSKGYLSALRTGWYTSVITIELSNIKENKCNGTDAKVKLIKQELDKYKNAVTELQLLMQSTPATNNRARRELPRFMNYTLNNAKKTNVTLSKKRKRRFLGFLLGVGSAIASGVAVSKVLHLEGEVNKIKSALLSTNKAVVSLSNGVSVLTSKVLDLKNYIDKQLLPIVNKQSCSISNIETVIEFQQKNNRLLEITREFSVNAGVTTPVSTYMLTNSELLSLINDMPITNDQKKLMSNNVQIVRQQSYSIMSIIKEEVLAYVVQLPLYGVIDTPCWKLHTSPLCTTNTKEGSNICLTRTDRGWYCDNAGSVSFFPQAETCKVQSNRVFCDTMNSLTLPSEVNLCNVDIFNPKYDCKIMTSKTDVSSSVITSLGAIVSCYGKTKCTASNKNRGIIKTFSNGCDYVSNKGVDTVSVGNTLYYVNKQEGKSLYVKGEPIINFYDPLVFPSDEFDASISQVNEKINQSLAFIRKSDELLHNVNAGKSTTNIMITTIIIVIIVILLSLIAVGLLLYCKARSTPVTLSKDQLSGINNIAFSN

SEQ ID NO: 2 - protein, 574 aa, Respiratory syncytial virus
MELLIHRLSAIFLTLAINALYLTSSQNITEEFYQSTCSAVSRGYFSALRTGWYTSVITIELSNIKETKCNGTDTKVKLIKQELDKYKNAVTELQLLMQNTPAANNRARREAPQYMNYTINTTKNLNVSISKKRKRRFLGFLLGVGSAIASGIAVSKVLHLEGEVNKIKNALLSTNKAVVSLSNGVSVLTSKVLDLKNYINNQLLPIVNQQSCRISNIETVIEFQQKNSRLLEINREFSVNAGVTTPLSTYMLTNSELLSLINDMPITNDQKKLMSSNVQIVRQQSYSIMSIIKEEVLAYVVQLPIYGVIDTPCWKLHTSPLCTTNIKEGSNICLTRTDRGWYCDNAGSVSFFPQADTCKVQSNRVFCDTMNSLTLPSEVSLCNTDIFNSKYDCKIMTSKTDISSSVITSLGAIVSCYGKTKCTASNKNRGIIKTFSNGCDYVSNKGVDTVSVGNTLYYVNKLEGKNLYVKGEPIINYYDPLVFPSDEFDASISQVNEKINQSLAFIRRSDELLHNVNTGKSTTNIMITTIIIVIIVVLLSLIAIGLLLYCKAKNTPVTLSKDQLSGINNIAFSK

SEQ ID NO: 3 - RNA, 1725 nt, Respiratory syncytial virus
  source 1..1725: mol_type = genomic RNA
atggagctgctgatccacaggttaagtgcaatcttcctaactcttgctattaatgcattgtacctcacctcaagtcagaacataactgaggagttttaccaatcgacatgtagtgcagttagcagaggttattttagtgctttaagaacaggttggtataccagtgtcataacaatagaattaagtaatataaaagaaaccaaatgcaatggaactgacactaaagtaaaacttataaaacaagaattagataagtataagaatgcagtgacagaattacagctacttatgcaaaacacaccagctgccaacaaccgggccagaagagaagcaccacagtatatgaactatacaatcaataccactaaaaacctaaatgtatcaataagcaagaagaggaaacgaagatttctgggcttcttgttaggtgtaggatctgcaatagcaagtggtatagctgtatccaaagttctacaccttgaaggagaagtgaacaagatcaaaaatgctttgttatctacaaacaaagctgtagtcagtctatcaaatggggtcagtgttttaaccagcaaagtgttagatctcaagaattacataaataaccaattattacccatagtaaatcaacagagctgtcgcatctccaacattgaaacagttatagaattccagcagaagaacagcagattgttggaaatcaacagagaattcagtgtcaatgcaggtgtaacaacacctttaagcacttacatgttaacaaacagtgagttactatcattgatcaatgatatgcctataacaaatgatcagaaaaaattaatgtcaagcaatgttcagatagtaaggcaacaaagttattctatcatgtctataataaaggaagaagtccttgcatatgttgtacagctacctatctatggtgtaatagatacaccttgctggaaattacacacatcacctctatgcaccaccaacatcaaagaaggatcaaatatttgtttaacaaggactgatagaggatggtattgtgataatgcaggatcagtatccttctttccacaggctgacacttgtaaagtacagtccaatcgagtattttgtgacactatgaacagtttgacattaccaagtgaagtcagcctttgtaacactgacatattcaattccaagtatgactgcaaaattatgacatcaaaaacagacataagcagctcagtaattacttctcttggagctatagtgtcatgctatggtaaaactaaatgcactgcatccaacaaaaatcgtgggattataaagacattttctaatggttgtgactatgtgtcaaacaaaggagtagatactgtgtcagtgggcaacactttatactatgtaaacaagctggaaggcaagaacctttatgtaaaaggggaacctataataaattactatgaccctctagtgtttccttctgatgagtttgatgcatcaatatctcaagtcaatgaaaaaatcaatcaaagtttagcttttattcgtagatctgatgaattactacataatgtaaatactggcaaatctactacaaatattatgataactacaattattatagtaatcattgtagtattgttatcattaatagctattggtttgctgttgtattgcaaagccaaaaacacaccagttacactaagcaaagaccaactaagtggaatcaataatattgcattcagcaaatag

SEQ ID NO: 4 - DNA, 1725 bp, synthetic construct
  misc_feature 1..1725: note = Recombinant RSV F
  source 1..1725: mol_type = other DNA
atggaactgctgatcctgaaggccaacgccatcacaacaatcctgaccgccgtgaccttctgcttcgccagcggccagaacatcaccgaggaattctaccagagcacctgtagcgccgtgtccaagggctacctgagcgccctgagaaccggctggtacaccagcgtgatcaccatcgagctgtccaacatcaaagaaaacaagtgcaacggcaccgacgccaaagtgaagctgatcaagcaggaactggacaagtacaagaacgccgtgaccgagctgcagctgctgatgcagtccacccccgccaccaacaaccgggccagaagagaactgccccggttcatgaactacaccctcaacaacgccaaaaagaccaacgtgaccctgagcaagaagcggaagcggcggttcctgggcttcctgctgggcgtgggcagcgccattgcctctggcgtggccgtgtctaaggtgctgcacctggaaggcgaagtgaacaagatcaagagcgccctgctgtccacaaacaaggccgtggtgtccctgagcaacggcgtgtccgtgctgacctccaaggtgctggatctgaagaactacatcgacaagcagctgctgcccatcgtgaacaagcagagctgcagcatcagcaacatcgagacagtgatcgagttccagcagaagaacaaccggctgctggaaatcacccgcgagttcagcgtgaacgccggcgtgaccacccccgtgtccacctacatgctgaccaacagcgagctgctgtccctgatcaatgacatgcccatcaccaacgaccagaaaaagctgatgagcaacaacgtgcagatcgtgcggcagcagagctactccatcatgagcatcatcaaagaagaggtgctggcctacgtggtgcagctgcccctgtacggcgtgatcgacaccccctgctggaagctgcacaccagccccctgtgcaccaccaacacaaaagagggcagcaacatctgcctgacccggaccgaccggggctggtactgcgataatgccggcagcgtgtcattctttccacaggccgagacatgcaaggtgcagagcaaccgggtgttctgcgacaccatgaacagcctgaccctgccctccgaagtgaacctgtgcaacgtggacatcttcaaccctaagtacgactgcaagatcatgaccagcaagaccgacgtgtccagctccgtgatcacctccctgggcgccatcgtgtcctgctacggcaagaccaagtgcaccgccagcaacaagaaccggggcatcatcaagaccttcagcaacggctgcgactacgtgtccaacaagggggtggacaccgtgtccgtgggcaacaccctgtactacgtgaacaaacaggaaggcaagagcctgtacgtgaagggcgagcccatcatcaacttctacgaccccctggtgttccccagcgacgagttcgacgccagcatcagccaggtcaacgagaagatcaaccagagcctggccttcatcagaaagagcgacgagctgctgcacaatgtgaatgccggcaagagcaccacaaacatcatgatcaccactatcatcatcgtgatcatcgtcatcctgctgagtctgatcgccgtgggcctgctgctgtactgcaaggccagatccacccctgtgaccctgtccaaggatcagctgtccggcatcaacaatatcgccttctccaactga

SEQ ID NO: 5 - DNA, 1725 bp, synthetic construct
  misc_feature 1..1725: note = Recombinant RSV F
  source 1..1725: mol_type = other DNA
atggaactgctgatcctgaaagccaacgctattactactatcctgaccgccgtgacattttgcttcgcatctggacagaacattactgaggaattctaccagtcaacatgcagcgccgtgtccaaaggatacctgagcgccctgcggaccggctggtatacatcagtgattactatcgagctgtccaacatcaaggaaaacaaatgtaatgggaccgacgcaaaggtgaaactgatcaagcaggagctggataagtacaaaaatgccgtgacagaactgcagctgctgatgcagtccacaccagcaactaacaatcgcgcccggagagagctgccccggttcatgaactataccctgaacaatgctaagaaaaccaatgtgacactgtccaagaaacgcaagaggcgcttcctgggatttctgctgggcgtggggtctgccatcgctagtggagtggccgtctctaaagtcctgcacctggagggcgaagtgaacaagatcaaaagcgccctgctgtccactaacaaggcagtggtcagtctgtcaaatggcgtgtccgtcctgacctctaaggtgctggacctgaaaaattatattgataagcagctgctgcctatcgtcaacaaacagagctgctccatttctaatatcgagacagtgatcgaattccagcagaagaacaatagactgctggagattaccagagagttcagcgtgaacgccggcgtcaccacacccgtgtccacctacatgctgacaaatagtgagctgctgtcactgattaacgacatgcctatcaccaatgatcagaagaaactgatgtccaacaatgtgcagatcgtcagacagcagagttactcaatcatgtctatcattaaggaggaagtcctggcctacgtggtccagctgccactgtatggcgtgatcgacaccccctgctggaaactgcatacatctcctctgtgcactaccaacacaaaggaaggaagtaatatctgcctgactcgaaccgaccggggatggtactgtgataacgcaggcagcgtgtccttctttccacaggccgagacctgcaaggtccagagcaacagggtgttctgtgacactatgaatagcctgaccctgccttccgaagtcaacctgtgcaatgtggacatctttaatccaaagtacgattgtaagatcatgactagcaagaccgatgtcagctcctctgtgattacttctctgggggccatcgtgagttgctacggaaagacaaaatgtactgccagcaacaaaaatcgcggcatcattaagaccttctccaacgggtgcgactatgtctctaacaagggcgtggatacagtgagtgtcgggaacactctgtactatgtcaataagcaggagggaaaaagcctgtacgtgaagggcgaacccatcattaacttctatgaccccctggtgttcccttccgacgagtttgatgcatctattagtcaggtgaacgaaaaaatcaatcagagtctggcctttattcggaagtcagatgagctgctgcacaacgtgaatgctggcaaatctacaactaacatcatgatcaccacaatcatcatcgtgattatcgtcattctgctgtcactgatcgctgtggggctgctgctgtactgtaaggcaagaagcaccccagtcactctgtcaaaagaccagctgtcagggattaacaacattgccttcagtaactga

SEQ ID NO: 6 - DNA, 1725 bp, synthetic construct; identical to SEQ ID NO: 4
  misc_feature 1..1725: note = Recombinant RSV F
  source 1..1725: mol_type = other DNA

SEQ ID NO: 7 - DNA, 1725 bp, synthetic construct; identical to SEQ ID NO: 5
  misc_feature 1..1725: note = Recombinant RSV F
  source 1..1725: mol_type = other DNA

SEQ ID NO: 8 - protein, 573 aa, synthetic construct
  REGION 1..573: note = Recombinant RSV F
MELLILKANAITTILTAVTFCFASGQNITEEFYQSTCSAVSKGYLSALRTGWYTSVITIELSNIKENKCNGTDAKVKLIKQELDKYKNAVTELQLLMQSTPATNNRARRELPRFMNYTLNNAKKTNVTLSKKRKRRFLGFLLGVGSAIASGVAVCKVLHLEGEVNKIKSALLSTNKAVVSLSNGVSVLTFKVLDLKNYIDKQLLPILNKQSCSISNIETVIEFQQKNNRLLEITREFSVNAGVTTPVSTYMLTNSELLSLINDMPITNDQKKLMSNNVQIVRQQSYSIMCIIKEEVLAYVVQLPLYGVIDTPCWKLHTSPLCTTNTKEGSNICLTRTDRGWYCDNAGSVSFFPQAETCKVQSNRVFCDTMNSLTLPSEVNLCNVDIFNPKYDCKIMTSKTDVSSSVITSLGAIVSCYGKTKCTASNKNRGIIKTFSNGCDYVSNKGVDTVSVGNTLYYVNKQEGKSLYVKGEPIINFYDPLVFPSDEFDASISQVNEKINQSLAFIRKSDELLHNVNAGKSTTNIMITTIIIVIIVILLSLIAVGLLLYCKYYRIQKRNRVDQNDKPYVLTNK

SEQ ID NO: 9 - DNA, 1722 bp, synthetic construct
  misc_feature 1..1722: note = Recombinant RSV F
  source 1..1722: mol_type = other DNA
atggaactgctgatcctgaaagccaacgctattactactatcctgaccgccgtgacattttgcttcgcatctggacagaacattactgaggaattctaccagtcaacatgcagcgccgtgtccaaaggatacctgagcgccctgcggaccggctggtatacatcagtgattactatcgagctgtccaacatcaaggaaaacaaatgtaatgggaccgacgcaaaggtgaaactgatcaagcaggagctggataagtacaaaaatgccgtgacagaactgcagctgctgatgcagtccacaccagcaactaacaatcgcgcccggagagagctgccccggttcatgaactataccctgaacaatgctaagaaaaccaatgtgacactgtccaagaaacgcaagaggcgcttcctgggatttctgctgggcgtggggtctgccatcgctagtggagtggccgtctgcaaagtcctgcacctggagggcgaagtgaacaagatcaaaagcgccctgctgtccactaacaaggcagtggtcagtctgtcaaatggcgtgtccgtcctgaccttcaaggtgctggacctgaaaaattatattgataagcagctgctgcctatcctgaacaaacagagctgctccatttctaatatcgagacagtgatcgaattccagcagaagaacaatagactgctggagattaccagagagttcagcgtgaacgccggcgtcaccacacccgtgtccacctacatgctgacaaatagtgagctgctgtcactgattaacgacatgcctatcaccaatgatcagaagaaactgatgtccaacaatgtgcagatcgtcagacagcagagttactcaatcatgtgcatcattaaggaggaagtcctggcctacgtggtccagctgccactgtatggcgtgatcgacaccccctgctggaaactgcatacatctcctctgtgcactaccaacacaaaggaaggaagtaatatctgcctgactcgaaccgaccggggatggtactgtgataacgcaggcagcgtgtccttctttccacaggccgagacctgcaaggtccagagcaacagggtgttctgtgacactatgaatagcctgaccctgccttccgaagtcaacctgtgcaatgtggacatctttaatccaaagtacgattgtaagatcatgactagcaagaccgatgtcagctcctctgtgattacttctctgggggccatcgtgagttgctacggaaagacaaaatgtactgccagcaacaaaaatcgcggcatcattaagaccttctccaacgggtgcgactatgtctctaacaagggcgtggatacagtgagtgtcgggaacactctgtactatgtcaataagcaggagggaaaaagcctgtacgtgaagggcgaacccatcattaacttctatgaccccctggtgttcccttccgacgagtttgatgcatctattagtcaggtgaacgaaaaaatcaatcagagtctggcctttattcggaagtcagatgagctgctgcacaacgtgaatgctggcaaatctacaactaacatcatgatcaccacaatcatcatcgtgattatcgtcattctgctgtcactgatcgctgtggggctgctgctgtactgtaagtactaccgtatccagaagaggaacagagttgaccagaacgataagccatacgtgctcactaacaagtga

SEQ ID NO: 10 - protein, 575 aa, synthetic construct
  REGION 1..575: note = Recombinant RSV F
MELLILKANAITTILTAVTFCFASGQNITEEFYQSTCSAVSKGYLSALRTGWYTSVITIELSNIKENKCNGTDAKVKLIKQELDKYKNAVTELQLLMQSTPATNNRARRELPRFMNYTLNNAKKTNVTLSKKRKRRFLGFLLGVGSAIASGVAVCKVLHLEGEVNKIKSALLSTNKAVVSLSNGVSVLTFKVLDLKNYIDKQLLPILNKQSCSISNIETVIEFQQKNNRLLEITREFSVNAGVTTPVSTYMLTNSELLSLINDMPITNDQKKLMSNNVQIVRQQSYSIMCIIKEEVLAYVVQLPLYGVIDTPCWKLHTSPLCTTNTKEGSNICLTRTDRGWYCDNAGSVSFFPQAETCKVQSNRVFCDTMNSLTLPSEVNLCNVDIFNPKYDCKIMTSKTDVSSSVITSLGAIVSCYGKTKCTASNKNRGIIKTFSNGCDYVSNKGVDTVSVGNTLYYVNKQEGKSLYVKGEPIINFYDPLVFPSDEFDASISQVNEKINQSLAFIRKSDELLHNVNAGKSTTNIMITTIIIILIMIIILFIINITIITIAIKYYRIQKRNRVDQNDKPYVLTNK

SEQ ID NO: 11 - DNA, 1728 bp, synthetic construct
  misc_feature 1..1728: note = Recombinant RSV F
  source 1..1728: mol_type = other DNA
atggaactgctgatcctgaaagccaacgctattactactatcctgaccgccgtgacattttgcttcgcatctggacagaacattactgaggaattctaccagtcaacatgcagcgccgtgtccaaaggatacctgagcgccctgcggaccggctggtatacatcagtgattactatcgagctgtccaacatcaaggaaaacaaatgtaatgggaccgacgcaaaggtgaaactgatcaagcaggagctggataagtacaaaaatgccgtgacagaactgcagctgctgatgcagtccacaccagcaactaacaatcgcgcccggagagagctgccccggttcatgaactataccctgaacaatgctaagaaaaccaatgtgacactgtccaagaaacgcaagaggcgcttcctgggatttctgctgggcgtggggtctgccatcgctagtggagtggccgtctgcaaagtcctgcacctggagggcgaagtgaacaagatcaaaagcgccctgctgtccactaacaaggcagtggtcagtctgtcaaatggcgtgtccgtcctgaccttcaaggtgctggacctgaaaaattatattgataagcagctgctgcctatcctgaacaaacagagctgctccatttctaatatcgagacagtgatcgaattccagcagaagaacaatagactgctggagattaccagagagttcagcgtgaacgccggcgtcaccacacccgtgtccacctacatgctgacaaatagtgagctgctgtcactgattaacgacatgcctatcaccaatgatcagaagaaactgatgtccaacaatgtgcagatcgtcagacagcagagttactcaatcatgtgcatcattaaggaggaagtcctggcctacgtggtccagctgccactgtatggcgtgatcgacaccccctgctggaaactgcatacatctcctctgtgcactaccaacacaaaggaaggaagtaatatctgcctgactcgaaccgaccggggatggtactgtgataacgcaggcagcgtgtccttctttccacaggccgagacctgcaaggtccagagcaacagggtgttctgtgacactatgaatagcctgaccctgccttccgaagtcaacctgtgcaatgtggacatctttaatccaaagtacgattgtaagatcatgactagcaagaccgatgtcagctcctctgtgattacttctctgggggccatcgtgagttgctacggaaagacaaaatgtactgccagcaacaaaaatcgcggcatcattaagaccttctccaacgggtgcgactatgtctctaacaagggcgtggatacagtgagtgtcgggaacactctgtactatgtcaataagcaggagggaaaaagcctgtacgtgaagggcgaacccatcattaacttctatgaccccctggtgttcccttccgacgagtttgatgcatctattagtcaggtgaacgaaaaaatcaatcagagtctggcctttattcggaagtcagatgagctgctgcacaacgtgaatgctggcaaatctacaactaacatcatgatcaccacaatcatcatcatcttgatcatgatcatcatcctgttcatcatcaacatcacaatcatcaccatcgctatcaagtactaccgtatccagaagaggaacagagttgaccagaacgataagccatacgtgctcactaacaagtga

SEQ ID NO: 12 - protein, 576 aa, synthetic construct
  REGION 1..576: note = Recombinant RSV F
MELLILKANAITTILTAVTFCFASGQNITEEFYQSTCSAVSKGYLSALRTGWYTSVITIELSNIKENKCNGTDAKVKLIKQELDKYKNAVTELQLLMQSTPATNNRARRELPRFMNYTLNNAKKTNVTLSKKRKRRFLGFLLGVGSAIASGVAVSKVLHLEGEVNKIKSALLSTNKAVVSLSNGVSVLTSKVLDLKNYIDKQLLPIVNKQSCSISNIETVIEFQQKNNRLLEITREFSVNAGVTTPVSTYMLTNSELLSLINDMPITNDQKKLMSNNVQIVRQQSYSIMSIIKEEVLAYVVQLPLYGVIDTPCWKLHTSPLCTTNTKEGSNICLTRTDRGWYCDNAGSVSFFPQAETCKVQSNRVFCDTMNSLTLPSEVNLCNVDIFNPKYDCKIMTSKTDVSSSVITSLGAIVSCYGKTKCTASNKNRGIIKTFSNGCDYVSNKGVDTVSVGNTLYYVNKQEGKSLYVKGEPIINFYDPLVFPSDEFDASISQVNEKINQSLAFIRKSDELLHNVNAGKSTTNIMITTITIIIVMIIILVIINITIIVVIIKFHRIQGKDQNDKNSEPYILTNRQ

SEQ ID NO: 13 - DNA, 1731 bp, synthetic construct
  misc_feature 1..1731: note = Recombinant RSV F
  source 1..1731: mol_type = other DNA
atggaactgctgatcctgaaggccaacgccatcaccaccatcctgaccgccgtgaccttctgctttgccagcggccagaacatcaccgaggaattctaccagagcacctgtagcgccgtgtccaagggctacctgagcgccctgagaaccggctggtacaccagcgtgatcaccatcgagctgagcaacatcaaagaaaacaagtgcaacggcaccgacgccaaagtgaagctgatcaagcaggaactggacaagtacaagaatgccgtgaccgaactgcagctgctgatgcagagcacccccgccaccaacaaccgggccagaagagaactgcccagattcatgaactacaccctgaacaacgccaaaaagaccaacgtgaccctgagcaagaagcggaagcggcggttcctgggctttctgctgggagtgggaagcgccattgctagcggagtggccgtgtctaaggtgctgcacctggaaggcgaagtgaacaagatcaagtccgccctgctgagcaccaacaaggccgtggtgtctctgagcaacggcgtgtccgtgctgaccagcaaggtgctggatctgaagaactacatcgacaaacagctgctgcccatcgtgaacaagcagagctgcagcatcagcaacatcgagacagtgatcgagttccagcagaagaacaaccggctgctggaaatcacccgcgagttcagcgtgaacgctggcgtgaccacccccgtgtccacctacatgctgaccaacagcgagctgctgtccctgatcaacgacatgcccatcaccaacgaccagaaaaagctgatgagcaacaacgtgcagatcgtgcggcagcagagctactccatcatgagcattatcaaagaagaggtgctggcctacgtggtgcagctgcctctgtacggcgtgatcgacaccccctgctggaagctgcacaccagccctctgtgcaccaccaacaccaaagagggctccaacatctgcctgacccggaccgacagaggctggtactgcgataatgccggctccgtctcattctttccacaagccgagacatgcaaggtgcagagcaaccgggtgttctgcgacaccatgaacagcctgaccctgccctccgaagtgaatctgtgcaacgtggacatcttcaaccctaagtacgactgcaagatcatgacctccaagaccgacgtgtccagctccgtgatcacaagcctgggcgccatcgtgtcctgctacggcaagaccaagtgcaccgccagcaacaagaaccggggcatcatcaagaccttcagcaacggctgcgactacgtgtccaacaagggggtggacaccgtgtctgtgggcaacaccctgtactacgtgaacaaacaggaaggcaagagcctgtacgtgaagggcgagcccatcatcaacttctacgaccccctggtgttccccagcgacgagttcgatgccagcatctcccaagtgaacgagaagatcaaccagagcctggccttcatcagaaagtccgatgagctgctgcacaatgtgaacgccggcaagtccaccaccaatatcatgatcaccacaatcaccatcatcattgtgatgattatcatcctcgtgatcatcaacatcacaatcatcgtcgtgattattaagttccaccggatccagggcaaggaccagaacgacaagaactccgagccctacatcctgacaaaccggcagtga

SEQ ID NO: 14 - protein, 576 aa, synthetic construct
  REGION 1..576: note = Recombinant RSV F
MELLILKANAITTILTAVTFCFASGQNITEEFYQSTCSAVSKGYLSALRTGWYTSVITIELSNIKENKCNGTDAKVKLIKQELDKYKNAVTELQLLMQSTPATNNRARRELPRFMNYTLNNAKKTNVTLSKKRKRRFLGFLLGVGSAIASGVAVCKVLHLEGEVNKIKSALLSTNKAVVSLSNGVSVLTSKVLDLKNYIDKQLLPIVNKQSCSISNIETVIEFQQKNNRLLEITREFSVNAGVTTPVSTYMLTNSELLSLINDMPITNDQKKLMSNNVQIVRQQSYSIMCIIKEEVLAYVVQLPLYGVIDTPCWKLHTSPLCTTNTKEGSNICLTRTDRGWYCDNAGSVSFFPQAETCKVQSNRVFCDTMNSLTLPSEVNLCNVDIFNPKYDCKIMTSKTDVSSSVITSLGAIVSCYGKTKCTASNKNRGIIKTFSNGCDYVSNKGVDTVSVGNTLYYVNKQEGKSLYVKGEPIINFYDPLVFPSDEFDASISQVNEKINQSLAFIRKSDELLHNVNAGKSTTNIMITTIIIVIIVILLSLIAVGLLLYCIIKFHRIQGKDQNDKNSEPYILTNRQ

SEQ ID NO: 15 - DNA, 1731 bp, synthetic construct
  misc_feature 1..1731: note = Recombinant RSV F
  source 1..1731: mol_type = other DNA
atggaactgctgatcctgaaggccaacgccatcaccaccatcctgaccgccgtgaccttctgctttgccagcggccagaacatcaccgaggaattctaccagagcacctgtagcgccgtgtccaagggctacctgagcgccctgagaaccggctggtacaccagcgtgatcaccatcgagctgagcaacatcaaagaaaacaagtgcaacggcaccgacgccaaagtgaagctgatcaagcaggaactggacaagtacaagaatgccgtgaccgaactgcagctgctgatgcagagcacccccgccaccaacaaccgggccagaagagaactgcccagattcatgaactacaccctgaacaacgccaaaaagaccaacgtgaccctgagcaagaagcggaagcggcggttcctgggctttctgctgggagtgggaagcgccattgctagcggagtggccgtgtgcaaggtgctgcacctggaaggcgaagtgaacaagatcaagtccgccctgctgagcaccaacaaggccgtggtgtctctgagcaacggcgtgtccgtgctgaccagcaaggtgctggatctgaagaactacatcgacaaacagctgctgcccatcgtgaacaagcagagctgcagcatcagcaacatcgagacagtgatcgagttccagcagaagaacaaccggctgctggaaatcacccgcgagttcagcgtgaacgctggcgtgaccacccccgtgtccacctacatgctgaccaacagcgagctgctgtccctgatcaacgacatgcccatcaccaacgaccagaaaaagctgatgagcaacaacgtgcagatcgtgcggcagcagagctactccatcatgtgcatcatcaaagaagaggtgctggcctacgtggtgcagctgcctctgtacggcgtgatcgacaccccctgctggaagctgcacaccagccctctgtgcaccaccaacaccaaagagggctccaacatctgcctgacccggaccgacagaggctggtactgcgataatgccggctccgtctcattctttccacaagccgagacatgcaaggtgcagagcaaccgggtgttctgcgacaccatgaacagcctgaccctgccctccgaagtgaatctgtgcaacgtggacatcttcaaccctaagtacgactgcaagatcatgacctccaagaccgacgtgtccagctccgtgatcacaagcctgggcgccatcgtgtcctgctacggcaagaccaagtgcaccgccagcaacaagaaccggggcatcatcaagaccttcagcaacggctgcgactacgtgtccaacaagggggtggacaccgtgtctgtgggcaacaccctgtactacgtgaacaaacaggaaggcaagagcctgtacgtgaagggcgagcccatcatcaacttctacgaccccctggtgttccccagcgacgagttcgatgccagcatctcccaagtgaacgagaagatcaaccagagcctggccttcatcagaaagtccgatgagctgctgcacaatgtgaacgccggcaagtccaccaccaatatcatgatcaccacaatcatcatcgtgattatcgtgatcctgctgagcctgatcgccgtgggcctgctgctgtactgtatcatcaagttccaccggatccagggcaaggaccagaacgacaagaactccgagccctacatcctgacaaaccggcagtga

SEQ ID NO: 16 - protein, 576 aa, synthetic construct
  REGION 1..576: note = Recombinant RSV F
MELLILKANAITTILTAVTFCFASGQNITEEFYQSTCSAVSKGYLSALRTGWYTSVITIELSNIKENKCNGTDAKVKLIKQELDKYKNAVTELQLLMQSTPATNNRARRELPRFMNYTLNNAKKTNVTLSKKRKRRFLGFLLGVGSAIASGVAVCKVLHLEGEVNKIKSALLSTNKAVVSLSNGVSVLTFKVLDLKNYIDKQLLPILNKQSCSISNIETVIEFQQKNNRLLEITREFSVNAGVTTPVSTYMLTNSELLSLINDMPITNDQKKLMSNNVQIVRQQSYSIMCIIKEEVLAYVVQLPLYGVIDTPCWKLHTSPLCTTNTKEGSNICLTRTDRGWYCDNAGSVSFFPQAETCKVQSNRVFCDTMNSLTLPSEVNLCNVDIFNPKYDCKIMTSKTDVSSSVITSLGAIVSCYGKTKCTASNKNRGIIKTFSNGCDYVSNKGVDTVSVGNTLYYVNKQEGKSLYVKGEPIINFYDPLVFPSDEFDASISQVNEKINQSLAFIRKSDELLHNVNAGKSTTNIMITTIIIVIIVILLSLIAVGLLLYCIIKFHRIQGKDQNDKNSEPYILTNRQ

SEQ ID NO: 17 - DNA, 1731 bp, synthetic construct
  misc_feature 1..1731: note = Recombinant RSV F
  source 1..1731: mol_type = other DNA
atggaactgctgatcctgaaggccaacgccatcaccaccatcctgaccgccgtgaccttctgctttgccagcggccagaacatcaccgaggaattctaccagagcacctgtagcgccgtgtccaagggctacctgagcgccctgagaaccggctggtacaccagcgtgatcaccatcgagctgagcaacatcaaagaaaacaagtgcaacggcaccgacgccaaagtgaagctgatcaagcaggaactggacaagtacaagaatgccgtgaccgaactgcagctgctgatgcagagcacccccgccaccaacaaccgggccagaagagaactgcccagattcatgaactacaccctgaacaacgccaaaaagaccaacgtgaccctgagcaagaagcggaagcggcggttcctgggctttctgctgggagtgggaagcgccattgctagcggagtggccgtgtgcaaggtgctgcacctggaaggcgaagtgaacaagatcaagtccgccctgctgagcaccaacaaggccgtggtgtctctgagcaacggcgtgtccgtgctgaccttcaaggtgctggatctgaagaactacatcgacaaacagctgctgcccatcttgaacaagcagagctgcagcatcagcaacatcgagacagtgatcgagttccagcagaagaacaaccggctgctggaaatcacccgcgagttcagcgtgaacgctggcgtgaccacccccgtgtccacctacatgctgaccaacagcgagctgctgtccctgatcaacgacatgcccatcaccaacgaccagaaaaagctgatgagcaacaacgtgcagatcgtgcggcagcagagctactccatcatgtgcatcatcaaagaagaggtgctggcctacgtggtgcagctgcctctgtacggcgtgatcgacaccccctgctggaagctgcacaccagccctctgtgcaccaccaacaccaaagagggctccaacatctgcctgacccggaccgacagaggctggtactgcgataatgccggctccgtctcattctttccacaagccgagacatgcaaggtgcagagcaaccgggtgttctgcgacaccatgaacagcctgaccctgccctccgaagtgaatctgtgcaacgtggacatcttcaaccctaagtacgactgcaagatcatgacctccaagaccgacgtgtccagctccgtgatcacaagcctgggcgccatcgtgtcctgctacggcaagaccaagtgcaccgccagcaacaagaaccggggcatcatcaagaccttcagcaacggctgcgactacgtgtccaacaagggggtggacaccgtgtctgtgggcaacaccctgtactacgtgaacaaacaggaaggcaagagcctgtacgtgaagggcgagcccatcatcaacttctacgaccccctggtgttccccagcgacgagttcgatgccagcatctcccaagtgaacgagaagatcaaccagagcctggccttcatcagaaagtccgatgagctgctgcacaatgtgaacgccggcaagtccaccaccaatatcatgatcaccacaatcatcatcgtgattatcgtgatcctgctgagcctgatcgccgtgggcctgctgctgtactgtatcatcaagttccaccggatccagggcaaggaccagaacgacaagaactccgagccctacatcctgacaaaccggcagtga

SEQ ID NO: 18 - DNA, 1728 bp, synthetic construct
  misc_feature 1..1728: note = Recombinant RSV F
  source 1..1728: mol_type = other DNA
atggaactgctgatcctgaaagccaacgctattactactatcctgaccgccgtgacattttgcttcgcatctggacagaacattactgaggaattctaccagtcaacatgcagcgccgtgtccaaaggatacctgagcgccctgcggaccggctggtatacatcagtgattactatcgagctgtccaacatcaaggaaaacaaatgtaatgggaccgacgcaaaggtgaaactgatcaagcaggagctggataagtacaaaaatgccgtgacagaactgcagctgctgatgcagtccacaccagcaactaacaatcgcgcccggagagagctgccccggttcatgaactataccctgaacaatgctaagaaaaccaatgtgacactgtccaagaaacgcaagaggcgcttcctgggatttctgctgggcgtggggtctgccatcgctagtggagtggccgtctgcaaagtcctgcacctggagggcgaagtgaacaagatcaaaagcgccctgctgtccactaacaaggcagtggtcagtctgtcaaatggcgtgtccgtcctgaccttcaaggtgctggacctgaaaaattatattgataagcagctgctgcctatcctgaacaaacagagctgctccatttctaatatcgagacagtgatcgaattccagcagaagaacaatagactgctggagattaccagagagttcagcgtgaacgccggcgtcaccacacccgtgtccacctacatgctgacaaatagtgagctgctgtcactgattaacgacatgcctatcaccaatgatcagaagaaactgatgtccaacaatgtgcagatcgtcagacagcagagttactcaatcatgtgcatcattaaggaggaagtcctggcctacgtggtccagctgccactgtatggcgtgatcgacaccccctgctggaaactgcatacatctcctctgtgcactaccaacacaaaggaaggaagtaatatctgcctgactcgaaccgaccggggatggtactgtgataacgcaggcagcgtgtccttctttccacaggccgagacctgcaaggtccagagcaacagggtgttctgtgacactatgaatagcctgaccctgccttccgaagtcaacctgtgcaatgtggacatctttaatccaaagtacgattgtaagatcatgactagcaagaccgatgtcagctcctctgtgattacttctctgggggccatcgtgagttgctacggaaagacaaaatgtactgccagcaacaaaaatcgcggcatcattaagaccttctccaacgggtgcgactatgtctctaacaagggcgtggatacagtgagtgtcgggaacactctgtactatgtcaataagcaggagggaaaaagcctgtacgtgaagggcgaacccatcattaacttctatgaccccctggtgttcccttccgacgagtttgatgcatctattagtcaggtgaacgaaaaaatcaatcagagtctggcctttattcggaagtcagatgagctgctgcacaacgtgaatgctggcaaatctacaactaacatcatgatcaccacaatcatcatcgtgattatcgtcattctgctgtcactgatcgctgtggggctgctgctgtactgtatcattaagttccaccggatccagggcaaggaccagaacgataaaaatagcgagccctacattctgaccaacagacag

SEQ ID NO: 19 - protein, 576 aa, synthetic construct
  REGION 1..576: note = Recombinant RSV F
MELLILKANAITTILTAVTFCFASGQNITEEFYQSTCSAVSKGYLSALRTGWYTSVITIELSNIKENKCNGTDAKVKLIKQELDKYKNAVTELQLLMQSTPATNNRARRELPRFMNYTLNNAKKTNVTLSKKRKRRFLGFLLGVGSAIASGVAVCKVLHLEGEVNKIKSALLSTNKAVVSLSNGVSVLTSKVLDLKNYIDKQLLPIVNKQSCSISNIETVIEFQQKNNRLLEITREFSVNAGVTTPVSTYMLTNSELLSLINDMPITNDQKKLMSNNVQIVRQQSYSIMCIIKEEVLAYVVQLPLYGVIDTPCWKLHTSPLCTTNTKEGSNICLTRTDRGWYCDNAGSVSFFPQAETCKVQSNRVFCDTMNSLTLPSEVNLCNVDIFNPKYDCKIMTSKTDVSSSVITSLGAIVSCYGKTKCTASNKNRGIIKTFSNGCDYVSNKGVDTVSVGNTLYYVNKQEGKSLYVKGEPIINFYDPLVFPSDEFDASISQVNEKINQSLAFIRKSDELLHNVNAGKSTTNIMITTITIIIVMIIILVIINITIIVVIIKFHRIQGKDQNDKNSEPYILTNRQ

SEQ ID NO: 20 - DNA, 1731 bp, synthetic construct
  misc_feature 1..1731: note = Recombinant RSV F
  source 1..1731: mol_type = other DNA
atggaactgctgatcctgaaggccaacgccatcaccaccatcctgaccgccgtgaccttctgctttgccagcggccagaacatcaccgaggaattctaccagagcacctgtagcgccgtgtccaagggctacctgagcgccctgagaaccggctggtacaccagcgtgatcaccatcgagctgagcaacatcaaagaaaacaagtgcaacggcaccgacgccaaagtgaagctgatcaagcaggaactggacaagtacaagaatgccgtgaccgaactgcagctgctgatgcagagcacccccgccaccaacaaccgggccagaagagaactgcccagattcatgaactacaccctgaacaacgccaaaaagaccaacgtgaccctgagcaagaagcggaagcggcggttcctgggctttctgctgggagtgggaagcgccattgctagcggagtggccgtgtgcaaggtgctgcacctggaaggcgaagtgaacaagatcaagtccgccctgctgagcaccaacaaggccgtggtgtctctgagcaacggcgtgtccgtgctgaccagcaaggtgctggatctgaagaactacatcgacaaacagctgctgcccatcgtgaacaagcagagctgcagcatcagcaacatcgagacagtgatcgagttccagcagaagaacaaccggctgctggaaatcacccgcgagttcagcgtgaacgctggcgtgaccacccccgtgtccacctacatgctgaccaacagcgagctgctgtccctgatcaacgacatgcccatcaccaacgaccagaaaaagctgatgagcaacaacgtgcagatcgtgcggcagcagagctactccatcatgtgcatcatcaaagaagaggtgctggcctacgtggtgcagctgcctctgtacggcgtgatcgacaccccctgctggaagctgcacaccagccctctgtgcaccaccaacaccaaagagggctccaacatctgcctgacccggaccgacagaggctggtactgcgataatgccggctccgtctcattctttccacaagccgagacatgcaaggtgcagagcaaccgggtgttctgcgacaccatgaacagcctgaccctgccctccgaagtgaatctgtgcaacgtggacatcttcaaccctaagtacgactgcaagatcatgacctccaagaccgacgtgtccagctccgtgatcacaagcctgggcgccatcgtgtcctgctacggcaagaccaagtgcaccgccagcaacaagaaccggggcatcatcaagaccttcagcaacggctgcgactacgtgtccaacaagggggtggacaccgtgtctgtgggcaacaccctgtactacgtgaacaaacaggaaggcaagagcctgtacgtgaagggcgagcccatcatcaacttctacgaccccctggtgttccccagcgacgagttcgatgccagcatctcccaagtgaacgagaagatcaaccagagcctggccttcatcagaaagtccgatgagctgctgcacaatgtgaacgccggcaagtccaccaccaatatcatgatcaccacaatcaccatcatcattgtgatgattatcatcctcgtgatcatcaacatcacaatcatcgtcgtgattattaagttccaccggatccagggcaaggaccagaacgacaagaactccgagccctacatcctgacaaaccggcagtga

SEQ ID NO: 21 - protein, 576 aa, synthetic construct
  REGION 1..576: note = Recombinant RSV F
MELLILKANAITTILTAVTFCFASGQNITEEFYQSTCSAVSKGYLSALRTGWYTSVITIELSNIKENKCNGTDAKVKLIKQELDKYKNAVTELQLLMQSTPATNNRARRELPRFMNYTLNNAKKTNVTLSKKRKRRFLGFLLGVGSAIASGVAVCKVLHLEGEVNKIKSALLSTNKAVVSLSNGVSVLTFKVLDLKNYIDKQLLPILNKQSCSISNIETVIEFQQKNNRLLEITREFSVNAGVTTPVSTYMLTNSELLSLINDMPITNDQKKLMSNNVQIVRQQSYSIMCIIKEEVLAYVVQLPLYGVIDTPCWKLHTSPLCTTNTKEGSNICLTRTDRGWYCDNAGSVSFFPQAETCKVQSNRVFCDTMNSLTLPSEVNLCNVDIFNPKYDCKIMTSKTDVSSSVITSLGAIVSCYGKTKCTASNKNRGIIKTFSNGCDYVSNKGVDTVSVGNTLYYVNKQEGKSLYVKGEPIINFYDPLVFPSDEFDASISQVNEKINQSLAFIRKSDELLHNVNAGKSTTNIMITTITIIIVMIIILVIINITIIVVIIKFHRIQGKDQNDKNSEPYILTNRQ

SEQ ID NO: 22 - DNA, 1731 bp, synthetic construct
  misc_feature 1..1731: note = Recombinant RSV F
  source 1..1731: mol_type = other DNA
atggaactgctgatcctgaaggccaacgccatcaccaccatcctgaccgccgtgaccttctgctttgccagcggccagaacatcaccgaggaattctaccagagcacctgtagcgccgtgtccaagggctacctgagcgccctgagaaccggctggtacaccagcgtgatcaccatcgagctgagcaacatcaaagaaaacaagtgcaacggcaccgacgccaaagtgaagctgatcaagcaggaactggacaagtacaagaatgccgtgaccgaactgcagctgctgatgcagagcacccccgccaccaacaaccgggccagaagagaactgcccagattcatgaactacaccctgaacaacgccaaaaagaccaacgtgaccctgagcaagaagcggaagcggcggttcctgggctttctgctgggagtgggaagcgccattgctagcggagtggccgtgtgcaaggtgctgcacctggaaggcgaagtgaacaagatcaagtccgccctgctgagcaccaacaaggccgtggtgtctctgagcaacggcgtgtccgtgctgaccttcaaggtgctggatctgaagaactacatcgacaaacagctgctgcccatcttgaacaagcagagctgcagcatcagcaacatcgagacagtgatcgagttccagcagaagaacaaccggctgctggaaatcacccgcgagttcagcgtgaacgctggcgtgaccacccccgtgtccacctacatgctgaccaacagcgagctgctgtccctgatcaacgacatgcccatcaccaacgaccagaaaaagctgatgagcaacaacgtgcagatcgtgcggcagcagagctactccatcatgtgcatcatcaaagaagaggtgctggcctacgtggtgcagctgcctctgtacggcgtgatcgacaccccctgctggaagctgcacaccagccctctgtgcaccaccaacaccaaagagggctccaacatctgcctgacccggaccgacagaggctggtactgcgataatgccggctccgtctcattctttccacaagccgagacatgcaaggtgcagagcaaccgggtgttctgcgacaccatgaacagcctgaccctgccctccgaagtgaatctgtgcaacgtggacatcttcaaccctaagtacgactgcaagatcatgacctccaagaccgacgtgtccagctccgtgatcacaagcctgggcgccatcgtgtcctgctacggcaagaccaagtgcaccgccagcaacaagaaccggggcatcatcaagaccttcagcaacggctgcgactacgtgtccaacaagggggtggacaccgtgtctgtgggcaacaccctgtactacgtgaacaaacaggaaggcaagagcctgtacgtgaagggcgagcccatcatcaacttctacgaccccctggtgttccccagcgacgagttcgatgccagcatctcccaagtgaacgagaagatcaaccagagcctggccttcatcagaaagtccgatgagctgctgcacaatgtgaacgccggcaagtccaccaccaatatcatgatcaccacaatcaccatcatcattgtgatgattatcatcctcgtgatcatcaacatcacaatcatcgtcgtgattattaagttccaccggatccagggcaaggaccagaacgacaagaactccgagccctacatcctgacaaaccggcagtga

SEQ ID NO: 23 - DNA, 1731 bp, synthetic construct
  misc_feature 1..1731: note = Recombinant RSV F
  source 1..1731: mol_type = other DNA
atggaactgctgatcctgaaagccaacgctattactactatcctgaccgccgtgacattttgcttcgcatctggacagaacattactgaggaattctaccagtcaacatgcagcgccgtgtccaaaggatacctgagcgccctgcggaccggctggtatacatcagtgattactatcgagctgtccaacatcaaggaaaacaaatgtaatgggaccgacgcaaaggtgaaactgatcaagcaggagctggataagtacaaaaatgccgtgacagaactgcagctgctgatgcagtccacaccagcaactaacaatcgcgcccggagagagctgccccggttcatgaactataccctgaacaatgctaagaaaaccaatgtgacactgtccaagaaacgcaagaggcgcttcctgggatttctgctgggcgtggggtctgccatcgctagtggagtggccgtctgcaaagtcctgcacctggagggcgaagtgaacaagatcaaaagcgccctgctgtccactaacaaggcagtggtcagtctgtcaaatggcgtgtccgtcctgaccttcaaggtgctggacctgaaaaattatattgataagcagctgctgcctatcctgaacaaacagagctgctccatttctaatatcgagacagtgatcgaattccagcagaagaacaatagactgctggagattaccagagagttcagcgtgaacgccggcgtcaccacacccgtgtccacctacatgctgacaaatagtgagctgctgtcactgattaacgacatgcctatcaccaatgatcagaagaaactgatgtccaacaatgtgcagatcgtcagacagcagagttactcaatcatgtgcatcattaaggaggaagtcctggcctacgtggtccagctgccactgtatggcgtgatcgacaccccctgctggaaactgcatacatctcctctgtgcactaccaacacaaaggaaggaagtaatatctgcctgactcgaaccgaccggggatggtactgtgataacgcaggcagcgtgtccttctttccacaggccgagacctgcaaggtccagagcaacagggtgttctgtgacactatgaatagcctgaccctgccttccgaagtcaacctgtgcaatgtggacatctttaatccaaagtacgattgtaagatcatgactagcaagaccgatgtcagctcctctgtgattacttctctgggggccatcgtgagttgctacggaaagacaaaatgtactgccagcaacaaaaatcgcggcatcattaagaccttctccaacgggtgcgactatgtctctaacaagggcgtggatacagtgagtgtcgggaacactctgtactatgtcaataagcaggagggaaaaagcctgtacgtgaagggcgaacccatcattaacttctatgaccccctggtgttcccttccgacgagtttgatgcatctattagtcaggtgaacgaaaaaatcaatcagagtctggcctttattcggaagtcagatgagctgctgcacaacgtgaatgctggcaaatctacaactaacatcatgatcaccacaatcaccatcattatcgtgatgattatcattctggtcatcattaacatcacaatcattgtggtcatcattaagttccaccggattcagggcaaggaccagaacgataaaaatagcgagccctacatcctgaccaatagacagtga

SEQ ID NO: 24 - protein, 524 aa, Human parainfluenza virus 1
MAGLLSTFDTFSSRRSESINKSGGGAIIPGQRSTVSVFTLGPSVTDDADKLLIATTFLAHSLDTDKQHSQRGGFLVSLLAMAYSSPELYLTTNGVNADVKYVIYNIERDPKRTKTDGFIVKTRDMEYERTTEWLFGPMINKNPLFQGQRENADLEALLQTYGYPACLGAIIVQVWIVLVKAITSSAGLRKGFFNRLEAFRQDGTVKSALVFTGDTVEGIGAVMRSQQSLVSLMVETLVTMNTSRSDLTTLEKNIQIVGNYIRDAGLASFMNTIKYGVETKMAALTLSNLRPDINKLRSLVDIYLSKGARAPFICILRDPVHGDFAPGNYPALWSYAMGVAVVQNKAMQQYVTGRTYLDMEMFLLGQAVAKDADSKISSALEEELGVTDTAKERLRHHLTNLSGGDGAYHKPTGGGAIEVAIDHTDITFGVEDTADRDNKNWTNDSNERWMNHSISNHTITIRGAEELEEETNDEDITDIENKIARRLADRKQRLSQANNKRDTSSDADYENDDDATAAAGIGGI

SEQ ID NO: 25 - protein, 568 aa, Human parainfluenza virus 1
MDQDAFFFERDPEAEGEAPRKQESLSDVIGLLDVVLSYKPTEIGEDRSWLHGIIDNPKENKPSCKADDNNKDRAISTSTQDHRSSEESGISRRTSESKTETHARILDQQGIHRASRRGTSPNPLPENMGNERNTRIDEDSPNERRHQRSVLTDEDRKMAENSNKREEDQVEGFPEEVRRSTPLSDDGEGRTNNNGRSMETSSTHSTRITDVITNPSPELEDAVLQRNKRRPTTIKRNQTRSERTQSSELHKSTSENSSNLEDHNTKTSPKVPPSKNEESAATPKNNHNHRKTRYTTNNANNNTKSPPTPEHDATANEEETSNTSVDEMAKLLVSLGVMKSQHEFELSRSASHVFAKRMLKSANYKEMTFNLCGMLISVEKSLENKVEENRTLLKQIQEEINSSRDLHKRFSEYQKEQNSLMMANLSTLHIITDRGGKTGNPSDTTRSPSVFTKGKDNKVKKTRFDPSMEALGGQEFKPDLIREDELRDDIKNPVLEENNNEPQASNASRLIPSTEKHTLHSLKLVIENSPLSRVEKKAYIKSLYKCRTNQEVKNVMELFEEDIDSLTN

SEQ ID NO: 26 - protein, 204 aa, Human parainfluenza virus 1
MPSFLRGILKPKERHHENKNHSQMSSDSLTSSYPTSPQKLEKTEAGSMVSSTTQKKTSHHAKPTITTKTEQSQRRPKIIDQVRRVESLGEQVSQKQRHMLESLINKVYTGPLGEELVQTLYLRIWAMKETPESTKILQMREDIRDQYLRMKTERWLRTLIRGKKTKLRDFQKRYEEVHPYLMMERVEQIIMEEAWKLAAHIVQE

SEQ ID NO: 27 - protein, 348 aa, Human parainfluenza virus 1
MAETYRFPRFSHEENGTVEPLPLKTGPDKKAIPHIRIVKVGDPPKHGVRYLDVLLLGFFETPKQGPLSGSISDLTESTSYSICGSGSLPIGIAKYYGTDQELLKACIDLKITVRRTVRSGEMIVYMVDSIHAPLLPWSSRLRQGMIYNANKVALAPQCLPVDKDIRFRVVFVNGTSLGTITIAKVPKTLADLALPNSISVNLLVTLRAGVSTEQKGILPVLDDDGEKKLNFMVHLGIIRRKVGKIYSVEYCKNKIEKMKLIFSLGLVGGISFHVHATGTLSKTLMSQLAWKKAVCYPLMDVNPHMNLVIWAASVEITSVDAVFQPAIPKEFRYYPNVVAKSIGKIRRI

SEQ ID NO: 28 - protein, 555 aa, Human parainfluenza virus 1
MQKSEILFLVYSSLLLSSSLCQIPVEKLSNVGVIINEGKLLKIAGSYESRYIVLSLVPSIDLQDGCGTTQIIQYKNLLNRLLIPLKDALDLQESLITITNDTTVTNDNPQTRFFGAVIGTIALGVATAAQITAGIALAEAREARKDIALIKDSIVKTHNSVELIQRGIGEQIIALKTLQDFVNDEIRPAIGELRCETTALKLGIKLTQHYSELATAFSSNLGTIGEKSLTLQALSSLYSANITEILSTTKKDKSDIYDIIYTEQVKGTVIDVDLEKYMVTLLVKIPILSEIPGVLIYRASSISYNIEGEEWHVAIPNYIINKASSLGGADVTNCIESKLAYICPRDPTQLIPDNQQKCILGDVSKCPVTKVINNLVPKFAFINGGVVANCIASTCTCGTNRIPVNQDRSRGVTFLTYTNCGLIGINGIELYANKRGRDTTWGNQIIKVGPAVSIRPVDISLNLASATNFLEESKTELMKARAIISAVGGWHNTESTQIIMIIIVCILIIIICGILYYLYRVRRLLVMINSTHNSPVNAYTLESRMRNPYMGNNSN

SEQ ID NO: 29 - protein, 575 aa, Human parainfluenza virus 1
MAEKGKTNSSYWSTTRNDNSTVNTHINTPAGRTHIWLLIATTMHTVLSFIIMILCIDLIIKQDTCMKTNIMTVSSMNESAKIIKETITELIRQEVISRTINIQSSVQSGIPILLNKQSRDLTQLIEKSCNRQELAQICENTIAIHHADGISPLDPHDFWRCPVGEPLLSNNPNISLLPGPSLLSGSTTISGCVRLPSLSIGDAIYAYSSNLITQGCADIGKSYQVLQLGYISLNSDMYPDLNPVISHTYDINDNRKSCSVIAAGTRGYQLCSLPTVNETTDYSSEGIEDLVFDILDLKGKTKSHRYKNEDITFDHPFSAMYPSVGSGIKIENTLIFLGYGGLTTPLQGDTKCVINRCTNVNQSVCNDALKITWLKKRQVVNVLIRINNYLSDRPKIVVETIPITQNYLGAEGRLLKLGKKIYIYTRSSGWHSNLQIGSLDINNPMTIKWAPHEVLSRPGNQDCNWYNRCPRECISGVYTDAYPLSPDAVNVATTTLYANTSRVNPTIMYSNTSEIINMLRLKNVQLEAAYTTTSCITHFGKGYCFHIVEINQTSLNTLQPMLFKTSIPKICKITS

SEQ ID NO: 30 - protein, 2223 aa, Human parainfluenza virus 1
MDKQESTQNSSDILYPECHLNSPIVKSKIAQLHVLLDINQPYDLKDNSIINITKYKIRNGGLSPRQIKIRSLGKILKQEIKDIDRYTFEPYPIFSLELLRLDIPEICDKIRSIFSVSDRLIRELSSGFQELWLNILRQLGCVEGKEGFDSLKDVDIIPDITDKYNKNTWYRPFLTWFSIKYDMRWMQKNKSGNHLDVSNSHNFLDCKSYILIIYRDLVIIINKLKLTGYVLTPELVLMYCDVVEGRWNMSSAGRLDKRSSKITCKGEELWELIDSLFPNLGEDVYNIISLLEPLSLALIQLDDPVTNLKGAFMRHVLTELHTILIKDNIYTDSEADSIMESLIKIFRETSIDEKAEIFSFFRTFGHPSLEAITAADKVRTHMYSSKKIILKTLYECHAIFCAIIINGYRERHGGQWPPCEFPNHVCLELKNAQGSNSAISYECAVDNYSSFIGFKFLKFIEPQLDEDLTIYMKDKALSPRKAAWDSVYPDSNLYYKVPESEETRRLIEVFINDNNFNPADIINYVESGEWLNDDSFNISYSLKEKEIKQEGRLFAKMTYKMRAVQVLAETLLAKGVGELFSENGMVKGEIDLLKRLTTLSVSGVPRSNSVYNNPILHEKLIKNMNKCNSNGYWDERKKSKNEFKAADSSTEGYETLSCFLTTDLKKYCLNWRFESTALFGQRCNEIFGFKTFFNWMHPILEKSTIYVGDPYCPVPDRMHKELQDHDDTGIFIHNPRGGIEGYCQKLWTLISISAIHLAAVKVGVRVSAMVQGDNQAIAVTSRVPVTQTYKQKKTHVYEEITRYFGALREVMFDIGHELKLNETIISSKMFVYSKRIYYDGKILPQCLKALTRCVFWSETLVDENRSACSNIATSIAKAIENGYSPILGYCIALFKTCQQVCISLGMTINPTITSTIKDQYFKGKNWLRCAILIPANIGGFNYMSTARCFVRNIGDPAVAALADLKRFIKAGLLDKQVLYRVMNQEPGDSSFLDWASDPYSCNLPHSQSITTIIKNVTARSVLQESPNPLLSGLFSESSSEEDLNLASFLMDRKAILPRVAHEILDNSLTGVREAIAGMLDTTKSLVRASVRRGGLSYSILRRLINYDLLQYETLTRTLRKPVKDNIEYEYMCSVELAIGLRQKMWFHLTYGRPIHGLETPDPLELLRGSFIEGSEICKFCRSEGNNPMYTWFYLPDNIDLDTLSNGSPAIRIPYFGSATDERSEAQLGYVKNLSKPAKAAIRIAMVYTWAYGTDEISWMEAALIAQTRANLSLENLKLLTPVSTSTNLSHRLRDTATQMKFSSATLVRASRFITISNDNMALKEAGESKDTNLVYQQIMLTGLSLFEFNMRYKQGSLSKPMILHLHLNNKCCIIESPQELNIPPRSTLDLEITQENNKLIYDPDPLKDIDLELFSKVRDVVHTIDMNYWSDDEIIRATSICTAMTIADTMSQLDRDNLKEMIALINDDDINSLITEFMVIDIPLFCSTFGGILINQFAYSLYGLNVRGRDEIWGYVIRIIKDTSHAVLKVLSNALSHPKIFKRFWDAGVVEPVYGPNLSNQDKILLAISVCEYSVDLFMRDWQEGIPLEIFICDNDPNIAEMRKLSFLARHLAYLCSLAEIAKEGPKLESMTSLERLESLKEYLELTFLDDPILRYSQLTGLVIKIFPSTLTYIRKSSIKVLRVRGIGIPEVLEDWDPDADSMLLDNITAEVQHNIPLKKNERTPFWGLRVSKSQVLRLRGYEEIKREERGRSGVGLTLPFDGRYLSHQLRLFGINSTSCLKALELTYLLNPLVNKDKDRLYLGEGAGAMLSCYDATLGPCMNYYNSGVNSCDLNGQRELNIYPSEVALVGKKLNNVTSLCQRVKVLFNGNPGSTWIGNDECETLIWNELQNNSIGFIHCDMEGGEHKCDQVVLHEHYSVIRIAYLVGDKDVILVSKIAPRLGTDWTKQLSLYLRYWRDVSLIVLKTSNPASTEMYLISKDPKSDIIEDSNTVLANLLPLSKEDSIKIEKWILVEKAKVHDWIVRELKEGSASSGMLRPYHQALQIFGFEPNLNKLCRDFLSTLNIVDTKNCIITFDRVLRDTIFEWTRIKDADKKLRLTGKYDLYPLRDSGKLKVISRRLVISWIALSMSTRLVTGSFPDIKFESRLQLGIVSISSREIKNLRVISKIVIDKFEDIIHSVTYRFLTKEIKILMKILGAVKLFGARQSTSADITNIDTSDSIQ

SEQ ID NO: 31 - protein, 59 aa, Human parainfluenza virus 1
QIIMIIIVCILIIIICGILYYLYRVRRLLVMINSTHNSPVNAYTLESRMRNPYMGNNSN

SEQ ID NO: 32 - protein, 543 aa, Human parainfluenza virus 2
MSSVLKTFERFTIQQELQEQSEDTPIPLETIRPTIRVFVINNNDPIVRSRLLFFNLRIIMSNTAREGHRAGALLSLLSLPSAAMSNHIKLAMHSPEASIDRVEITGFENNSFRVIPDARSTMSRGEVLAFEALAEDIPDTLNHQTPFVNNDVEDDIFDETEKFLDVCYSVLMQAWIVTCKCMTAPDQPPVSVAKRMAKYQQQGRINARYVLQPEAQRLIQNAIRKSMVVRHFMTYELQLSQSRSLLANRYYAMVGDIGKYIEHSGMGGFFLTLKYGLGTRWPTLALAAFSGELQKLKALMLHYQSLGPMAKYMALLESPKLMDFVPSEYPLVYSYAMGIGTVLDTNMRNYAYGRSYLNPQYFQLGVETARKQQGAVDNRTAEDLGMTAADKADLTATISKLSLSQLPRGRQPISDPFAGANDRETGGQATDTPVYNFNPINNRRYDNYDSDSEDRIDNDQDQAIRENRGEPGQPNNQTSENQQRLNLPVPQRTSGMSSEEFQHSMNQYIRAMHEQYRGSQDDDANDATDGNDISLELVGDFDS

SEQ ID NO: 33 - protein, 395 aa, Human parainfluenza virus 2
MAEEPTYTTEQVDELIHAGLGTVDFFLSRPIDAQSSLGKGSIPPGVTAVLTNAAEAKSKPVAAGPVKPRRKKVISNTTPYTIADNIPPEKLPINTPIPNPLLPLARPHGKMTDIDIVTGNITEGSYKGVELAKLGKQTLLTRFTSNEPVSSAGSAQDPNFKRGGELIEKEQEATIGENGVLHGSEIRSKSSSGVIPGVPQSRLQLASSPAHVDPAPASAENVKEIIELLKGLDLRLQTVEGKVDKILATSATIINLKNEMTSLKASVATVEGMITTIKIMDPSTPTNVPVEEIRKSLHNVPVVIAGPTSGGFTAEGSDMISMDELARPTLSSTKKITRKPESKKDLTGIKLTLMQLANDCISRPDTKTEFVTKIQAATTESQLNEIKRSIIRSAI

SEQ ID NO: 34 - protein, 225 aa, Human parainfluenza virus 2
MAEEPTYTTEQVDELIHAGLGTVDFFLSRPIDAQSSLGKGSIPPGVTAVLTNAAEAKSKPVAAGPVKPRRKKVISNTTPYTIADNIPPEKLPINTPIPNPLLPLARPHGKMTDIDIVTGNITEGSYKGVELAKLGKQTLLTRFTSNEPVSSAGSAQDPNFKRGGANRERARGNHRREWSIAWVGDQVKVFEWCNPRCAPVTASARKFTCTCGSCPSICGECEGDH

SEQ ID NO: 35 - protein, 377 aa, Human parainfluenza virus 2
MPIISLPADPTSPSQSLTPFPIQLDTKDGKAGKLLKQIRIRYLNEPNSRHTPITFINTYGFVYARDTSGGIHSEISSDLAAGSITACMMTLGPGPNIQNANLVLRSLNEFYVKVKKTSSQREEAVFELVNIPTLLREHALCKRKTLVCSAEKFLKNPSKLQAGFEYVYIPTFVSITYSPRNLNYQVARPILKFRSRFVYSIHLELILRLLCKSDSPLMKSYNADRTGRGCLASVWIHVCNILKNKSIKQQGRESYFIAKCMSMQLQVSIADLWGPTIIIKSLGHIPKTALPFFSKDGIACHPLQDVSPTLTKSLWSVGCEIESAKLILQESDINELMGHQDLITDKIAIRSGQRTFERSKFSPFKKYASIPNLEAIN

SEQ ID NO: 36 - protein, 551 aa, Human parainfluenza virus 2
MHHLHPMIVCIFVMYTGIVGSDAIAGDQLLNVGVIQSKIRSLMYYTDGGASFIVVKLLPNLPPSNGTCNITSLDAYNVTLFKLLTPLIENLSKISAVTDTKPRRERFAGVVIGLAALGVATAAQITAAVAIVKANANAAAINNLASSIQSTNKAVSDVITASRTIATAVQAIQDHINGAIVNGITSASCRAHDALIGSILNLYLTELTTIFHNQITNPALTPLSIQALRILLGSTLPIVIESKLNTKLNTAELLSSGLLTGQIISISPMYMQMLIQINVPTFIMQPGAKVIDLIAISANHKLQEVVVQVPNRILEYANELQNYPANDCVVTPNSVFCRYNEGSPIPESQYQCLRGNLNSCTFTPIIGNFLKRFAFANGVLYANCKSLLCKCADPPHVVSQDDNQGISIIDIKRCSEMMLDTFSFRITSTFNATYVTDFSMINANIVHLSPLDLSNQINSINKSLKSAEDWIADSNFFANQARTAKTLYSLSAIALILSVITLVVVGLLIAYIIKLVSQIHQFRALAATTMFHRENPAVFSKNNHGNIYGIS

SEQ ID NO: 37 - protein, 571 aa, Human parainfluenza virus 2
MEDYSNLSLKSIPKRTCRIIFRTATILGICTLIVLCSSILHEIIHLDVSSGLMNSDESQQGIIQPIIESLKSLIALANQILYNVAIVIPLKIDSIETVILSALKDMHTGSMSNANCTPGNLLLHDAAYINGINKFLVLESYNGTPKYGPLLNIPSFIPSATSPHGCTRIPSFSLIKTHWCYTHNVMLGDCLDFTASNQYLSMGIIQQSAAGFPIFRTMKTIYLSDGINRKSCSVTAIPGGCVLYCYVATRSEKEDYATTDLAELRLAFYYYNDTFIERVISLPNTTGQWATINPAVGSGIYHLGFILFPVYGGLINGTTSYNEQSSRYFIPKHPNITCAGNSSKQAAIARSSYVIRYHSNRLIQSAVLICPLSDMHTEECNLVMFNNSQVMMGAEGRLYVIGNNLYYYQRSSSWWSASLFYRINTDFSKGIPPIIEAQWVPSYQVPRPGVMPCNATSFCPANCITGVYADVWPLNDPELMSRNALNPNYRFAGAFLKNESNRTNPTFYTASANSLLNTTGFNNTNHKAAYTSSTCFKNTGTQKIYCLIIIEMGSSLLGEFQIIPFLRELML

SEQ ID NO: 38 - protein, 2263 aa, Human parainfluenza virus 2
MAASSEILLPEVHLNSPIVKHKLIYYLLLGHFPHDLDISEISPLHNNDWDQIAREESNLAERLGVAKSELIKRVPAFRATRWRSHAAVLIWPSCIPFLVKFLPHSKLQPIEQWYKLINASCNTISDSIDRCMENISIKLTGKNNLFSRSRGTAGAGKNSKITLNDIQSIWESNKWQPNVSLWLTIKYQMRQLIMHQSSRQPTDLVHIVDTRSGLIVITPELVICFDRLNNVLMYFTFEMTLMVSDMFEGRMNVAALCTISHYLSPLGPRIDRLFSIVDELAQLLGDTVYKIIASLESLVYGCLQLKDPVVELTGSFHSFITQEIIDILIGSKALDKDESITVTTQLLDIFSNLSPDLIAEMLCLMRLWGHPTLTAAQAAGKVRESMCAGKLLDFPTIMKTLAFFHTILINGYRRKKNGMWPPLILPKNASKSLIEFQHDNAEISYEYTLKHWKEISLIEFRKCFDFDPGEELSIFMKDKAISAPKSDWMSVFRRSLIKQRHQRHHIPMPNPFNRRLLLNFLEDDSFDPVAELQYVTSGEYLRDDTFCASYSLKEKEIKPDGRIFAKLTNRMRSCQVIAEAILANHAGTLMKENGVVLNQLSLTKSLLTMSQIGIISEKAKRYTRDNISSQGFHTIKTDSKNKKKSKIASSYLTDPDDTFELSACFITTDLAKYCLQWRYQTIIHFARTLNRMYGVPHLFEWIHLRLIRSTLYVGDPFNPPATTDAFDLDKVLNGDIFIVSPKGGIEGLCQKMWTMISISVIILSSAESKTRVMSMVQGDNQAIAVTTRVPRSLPSVQKKELAYAASKLFFERLRANNYGLGHQLKAQETIISSTFFIYSKRVFYQGRILTQALKNASKLCLTADVLGECTQASCSNSATTIMRLTENGVEKDTCYKLNIYQSIRQLTYDLIFPQYSIPGETISEIFLQHPRLISRIVLLPSQLGGLNYLACSRLFNRNIGDPLGTAVADLKRLIKCGALESWILYNLLARKPGKGSWATLAADPYSLNQEYLYPPTTILKRHTQNTLMEICRNPMLKGVFTDNAKEEENLLAKFLLDRDIVLPRVAHIIIDQSSIGRKKQIQGFFDTTRTIMRRSFEIKPLSTKKTLSVIEYNTNYLSYNYPVILNPLPIPGYLNYITDQTCSIDISRSLRKLSWSSLLNGRTLEGLETPDPIEVVNGSLIVGTGDCDFCMQGDDKFTWFFLPMGIIIDGNPETNPPIRVPYIGSRTEERRVASMAYIKGATHSLKAALRGAGVYIWAFGDTVVNWNDALDIANTRVKISLEQLQTLTPLPTSANITHRLDDGATTLKFTPASSYAFSSYTHISNDQQYLEIDQRVVDSNIIYQQLMITGLGIIETYHNPPIRTSTQEITLHLHTSSSCCVRSVDGCLICESNGEVPQITVPYTNSFVYDPDPLADYEIAHLDYLSYQAKIGSTDYYSLTDKIDLLAHLTAKQMINSIIGLDETVSIVNDAVILSDYTNNWISECSYTKIDLVFKLMAWNFLLELAFQMYYLRISSWTNIFDYTYMTLRRIPGTALNNIAATISHPKLLRRAMNLDIITPIHAPYLASLDYVKLSIDAIQWGVKQVLADLSNGIDLEILILSEDSMEISDRAMNLIARKLTLLALVKGENYTFPKIKGMPPEEKCLVLTEYLAMCYQNTHHLDPDLQKYLYNLTNPKLTAFPSNNFYLTRKILNQIRESDEGQYIITSYYESFEQLETDIILHSTLTAPYDNSETLTKFDLSLDIFPHPESLEKYPLPVDHDSQSAISTLIPGPPSHHVLRPLGVSSTAWYKGISYCRYLETQKIQTGDHLYLAEGSGASMSLLELLFPGDTVYYNSLFSSGENPPQRNYAPLPTQFVQSVPYKLWQADLADDSNLIKDFVPLWNGNGAVTDLSTKDAVAFIIHKVGAEKASLVHIDLESTANINQQTLSRSQIHSLIIATTVLKRGGILVYKTSWLPFSRFSQLASLLWCFFDRIHLIRSSYSDPHSHEVYLVCRLAADFRTIGFSAALVTATTLHNDGFTTIHPDVVCSYWQHHLENVGRVEKVIDEILDGLATNFFAGDNGLILRCGGTPSSRKWLEIDQLASFDSVQDALVTLITIHLKEIIEVQSSHTEDYTSLLFTPYNIGAAGKVRTIIKLILERSLMYTVRNWLVLPSSIRDSVRQDLELGSFRLMSILSEQTFLKKTPTKKYLLDQLTRTYISTFFNSHSVLPLHRPYQKQIWKALGSVIYCSETVDIPLIRDIQIEDINDFEDIERGIDGEEL

SEQ ID NO: 39 - protein, 66 aa, Human parainfluenza virus 2
TLYSLSAIALILSVITLVVVGLLIAYIIKLVSQIHQFRALAATTMFHRENPAVFSKNNHGNIYGIS

SEQ ID NO: 40 - protein, 515 aa, Human parainfluenza virus 3
MLSLFDTFNARRQENITKSAGGAIIPGQKNTVSIFALGPTITDDNEKMTLALLFLSHSLDNEKQHAQRAGFLVSLLSMAYANPELYLTTNGSNADVKYVIYMIEKDLKRQKYGGFVVKTREMIYEKTTDWIFGSDLDYDQETMLQNGRNNSTIEDLVHTFGYPSCLGALIIQIWIVLVKAITSISGLRKGFFTRLEAFRQDGTVQAGLVLSGDTVDQIGSIMRSQQSLVTLMVETLITMNTSRNDLTTIEKNIQIVGNYIRDAGLASFFNTIRYGIETRMAALTLSTLRPDINRLKALMELYLSKGPRAPFICILRDPIHGEFAPGNYPAIWSYAMGVAVVQNRAMQQYVTGRSYLDIDMFQLGQAVARDAEAQMSSTLEDELGVTHESKESLKRHIRNINSSETSFHKPTGGSAIEMAIDEEPEQFEHRADQEQNGEPQSSIIQYAWAEGNRSDDQTEQATESDNIKTEQQNIRDRLNKRLNDKKKQSSQPPTNPTNRTNQDEIDDLFNAFGSN

SEQ ID NO: 41 - protein, 603 aa, Human parainfluenza virus 3
MESDAKNYQIMDSWEEESRDKSTNISSALNIIEFILSTDPQEDLSENDTINTRTQQLSATICQPEIKPTETSEKDSGSTDKNRQSGSSHECTTEAKDRNIDQETVQRGPGRRSSSDSRAETVVSGGIPRSITDSKNGTQNTEDIDLNEIRKMDKDSIEGKMRQSANVPSEISGSDDIFTTEQSRNSDHGRSLESISTPDTRSISVVTAATPDDEEEILMKNSRTKKSSSTHQEDDKRIKKGGKGKDWFKKSKDTDNQIPTSDYRSTSKGQKKISKTTTTNTDTKGQTEIQTESSETQSSSWNLIIDNNTDRNEQTSTTPPTTTSRSTYTKESIRTNSESKPKTQKTNGKERKDTEESNRFTERAITLLQNLGVIQSTSKLDLYQDKRVVCVANVLNNVDTASKIDFLAGLVIGVSMDNDTKLTQIQNEMLNLKADLKKMDESHRRLIENQREQLSLITSLISNLKIMTERGGKKDQNESNERVSMIKTKLKEEKIKKTRFDPLMEAQGIDKNIPDLYRHAGDTLENDVQVKSEILSSYNESNATRLIPKKVSSTMRSLVAVINNSNLSQSTKQSYINELKRCKNDEEVSELMDMFNEDVNNCQ

SEQ ID NO: 42 - protein, 353 aa, Human parainfluenza virus 3
MSITNSAIYTFPESSFSENGHIEPLPLKVNEQRKAVPHIRVAKIGNPPKHGSRYLDVFLLGFFEMERIKDKYGSVNDLDSDPSYKVCGSGSLPIGLAKYTGNDQELLQAATKLDIEVRRTVKAKEMVVYTVQNIKPELYPWSNRLRKGMLFDANKVALAPQCLPLDRSIKFRVIFVNCTAIGSITLFKIPKSMASLSLPNTISINLQVHIKTGVQTDSKGIVQILDEKGEKSLNFMVHLGLIKRKVGRMYSVEYCKQKIEKMRLIFSLGLVGGISLHVNATGSISKTLASQLVFKREICYPLMDLNPHLNLVIWASSVEITRVDAIFQPSLPGEFRYYPNIIAKGVGKIKQWN

SEQ ID NO: 43 - protein, 539 aa, Human parainfluenza virus 3
MPTSILLIITTMIMASFCQIDITKLQHVGVLVNSPKGMKISQNFETRYLILSLIPKIEDSNSCGDQQIKQYKKLLDRLIIPLYDGLRLQKDVIVTNQESNENTDPRTKRFFGGVIGTIALGVATSAQITAAVALVEAKQARSDIEKLKEAIRDTNKAVQSVQSSIGNLIVAIKSVQDYVNKEIVPSIARLGCEAAGLQLGIALTQHYSELTNIFGDNIGSLQEKGIKLQGIASLYRTNITEIFTTSTVDKYDIYDLLFTESIKVRVIDVDLNDYSITLQVRLPLLTRLLNTQIYKVDSISYNIQNREWYIPLPSHIMTKGAFLGGADVKECIEAFSSYICPSDPGFVLNHEIESCLSGNISQCPRTTVTSDIVPRYAFVNGGVVANCITTTCTCNGIGNRINQPPDQGVKIITHKECSTIGINGMLFNTNKEGTLAFYTPNDITLNNSVALDPIDISIELNKAKSDLEESKEWIRRSNQKLDSIGNWHQSSTTIIIILIMIIILFIINITIITIAIKYYRIQKRNRVDQNDKPYVLTNK

SEQ ID NO: 44 - protein, 572 aa, Human parainfluenza virus 3
MEYWKHTNHGKDAGNELETSMATHGNKLTNKIIYILWTIILVLLSIVFIIVLINSIKSEKAHESLLQDINNEFMEITEKIQMASDNTNDLIQSGVNTRLLTIQSHVQNYIPISLTQQMSDLRKFISEITIRNDNQEVLPQRITHDVGIKPLNPDDFWRCTSGLPSLMKTPKIRLMPGPGLLAMPTTVDGCVRTPSLVINDLIYAYTSNLITRGCQDIGKSYQVLQIGIITVNSDLVPDLNPRISHTFNINDNRKSCSLALLNTDVYQLCSTPKVDERSDYASSGIEDIVLDIVNYDGSISTTRFKNNNISFDQPYAALYPSVGPGIYYKGKIIFLGYGGLEHPINENVICNTTGCPGKTQRDCNQASHSPWFSDRRMVNSIIVVDKGLNSIPKLKVWTISMRQNYWGSEGRLLLLGNKIYIYTRSTSWHSKLQLGIIDITDYSDIRIKWTWHNVLSRPGNNECPWGHSCPDGCITGVYTDAYPLNPTGSIVSSVILDSQKSRVNPVITYSTATERVNELAILNRTLSAGYTTTSCITHYNKGYCFHIVEINHKSLNTFQPMLFKTEIPKSCS

SEQ ID NO: 45 - protein, 2233 aa, Human parainfluenza virus 3
MDTESNNGTVSDILYPECHLNSPIVKGKIAQLHTIMSLPQPYDMDDDSILVITRQKIKLNKLDKRQRSIRRLKLILTEKVNDLGKYTFIRYPEMSKEMFKLYIPGINSKVTELLLKADRTYSQMTDGLRDLWINVLSKLASKNDGSNYDLNEEINNISKVHTTYKSDKWYNPFKTWFTIKYDMRRLQKARNEITFNVGKDYNLLEDQKNFLLIHPELVLILDKQNYNGYLITPELVLMYCDVVEGRWNISACAKLDPKLQSMYQKGNNLWEVIDKLFPIMGEKTFDVISLLEPLALSLIQTHDPVKQLRGAFLNHVLSEMELIFESRESIKEFLSVDYIDKILDIFNKSTIDEIAEIFSFFRTFGHPPLEASIAAEKVRKYMYIGKQLKFDTINKCHAIFCTIIINGYRERHGGQWPPVTLPDHAHEFIINAYGSNSAISYENAVDYYQSFIGIKFNKFIEPQLDEDLTIYMKDKALSPKKSNWDTVYPASNLLYRTNASNESRRLVEVFIADSKFDPHQILDYVESGDWLDDPEFNISYSLKEKEIKQEGRLFAKMTYKMRATQVLSETLLANNIGKFFQENGMVKGEIELLKRLTTISISGVPRYNEVYNNSKSHTDDLKTYNKISNLNLSSNQKSKKFEFKSTDIYNDGYETVSCFLTTDLKKYCLNWRYESTALFGETCNQIFGLNKLFNWLHPRLEGSTIYVGDPYCPPSDKEHISLEDHPDSGFYVHNPRGGIEGFCQKLWTLISISAIHLAAVRIGVRVTAMVQGDNQAIAVTTRVPNNYDYRVKKEIVYKDVVRFFDSLREVMDDLGHELKLNETIISSKMFIYSKRIYYDGRILPQALKALSRCVFWSETVIDETRSASSNLATSFAKAIENGYSPVLGYACSIFKNIQQLYIALGMNINPTITQNIRDQYFRNPNWMQYASLIPASVGGFNYMAMSRCFVRNIGDPSVAALADIKRFIKANLLDRSVLYRIMNQEPGESSFLDWASDPYSCNLPQSQNITTMIKNITARNVLQDSPNPLLSGLFTNTMIEEDEELAEFLMDRKVILPRVAHDILDNSLTGIRNAIAGMLDTTKSLIRVGINRGGLTYSLLRKISNYDLVQYETLSRTLRLIVSDKIKYEDMCSVDLAIALRQKMWIHLSGGRMISGLETPDPLELLSGVVITGSEHCKICYSSDGTNPYTWMYLPGNIKIGSAETGISSLRVPYFGSVTDERSEAQLGYIKNLSKPAKAAIRIAMIYTWAFGNDEISWMEASQIAQTRANFTLDSLKILTPVATSTNLSHRLKDTATQMKFSSTSLIRVSRFITMSNDNMSIKEANETKDTNLIYQQIMLTGLSVFEYLFRLKETTGHNPIVMHLHIEDECCIKESFNDEHINPESTLELIRYPESNEFIYDKDPLKDVDLSKLMVIKDHSYTIDMNYWDDTDIIHAISICTAITIADTMSQLDRDNLKEIIVIANDDDINSLITEFLTLDILVFLKTFGGLLVNQFAYTLYSLKIEGRDLIWDYIMRTLRDTSHSILKVLSNALSHPKVFKRFWDCGVLNPIYGPNTASQDQIKLALSICEYSLDLFMREWLNGVSLEIYICDSDMEVANDRKQAFISRHLSFVCCLAEIASFGPNLLNLTYLERLDLLKQYLELNIKEDPTLKYVQISGLLIKSFPSTVTYVRKTAIKYLRIRGISPPEVIDDWDPVEDENMLDNIVKTINDNCNKDNKGNKINNFWGLALKNYQVLKIRSITSDSDDNDRLDANTSGLTLPQGGNYLSHQLRLFGINSTSCLKALELSQILMKEVNKDKDRLFLGEGAGAMLACYDATLGPAVNYYNSGLNITDVIGQRELKIFPSEVSLVGKKLGNVTQILNRVKVLFNGNPNSTWIGNMECESLIWSELNDKSIGLVHCDMEGAIGKSEETVLHEHYSVIRITYLIGDDDVVLVSKIIPTITPNWSRILYLYKLYWKDVSIISLKTSNPASTELYLISKDAYCTIMEPSEIVLSKLKRLSLLEENNLLKWIILSKKRNNEWLHHEIKEGERDYGIMRPYHMALQIFGFQINLNHLAKEFLSTPDLTNINNIIQSFQRTIKDVLFEWINITHDDKRHKLGGRYNIFPLKNKGKLRLLSRRLVLSWISLSLSTRLLTGRFPDEKFEHRAQTGYVSLADTDLESLKLLSKNIIKNYRECIGSISYWFLTKEVKILMKLIGGAKLLGIPRQYKEPEDQLLENYNQHDEFDID

SEQ ID NO: 46 - protein, 46 aa, Human parainfluenza virus 3
IIIILIMIIILFIINITIITIAIKYYRIQKRNRVDQNDKPYVLTNK

SEQ ID NO: 47 - protein, 515 aa, Bovine parainfluenza virus 3
MLSLFDTFSARRQENITKSAGGAVIPGQKNTVSIFALGPSITDDNDKMTLALLFLSHSLDNEKQHAQRAGFLVSLLSMAYANPELYLTSNGSNADVKYVIYMIEKDPGRQKYGGFVVKTREMVYEKTTDWMFGSDLEYDQDNMLQNGRSTSTIEDLVHTFGYPSCLGALIIQVWIILVKAITSISGLRKGFFTRLEAFRQDGTVKSSLVLSGDAVEQIGSIMRSQQSLVTLMVETLITMNTGRNDLTTIEKNIQIVGNYIRDAGLASFFNTIRYGIETRMAALTLSTLRPDINRLKALIELYLSKGPRAPFICILRDPVHGEFAPGNYPALWSYAMGVAVVQNKAMQQYVTGRSYLDIEMFQLGQAVARDAESQMSSILEDELGVTQEAKQSLKKHMKNISSSDTTFHKPTGGSAIEMAIDEEAGQPESRGDQDQGDEPRSSIVPYAWADETGNDNQTESTTEIDSIKTEQRNIRDRLNKRLNEKRKQSDPRSTDITNNTNQTEIDDLFSAFGSN

SEQ ID NO: 48 - protein, 596 aa, Bovine parainfluenza virus 3
MEDNVQNNQIMDSWEEGSGDKSSDISSALDIIEFILSTDSQENTADSNEINTGTTRLSTTIYQPESKTTETSKENSGPANKNRQFGASHERATETKDRNVNQETVQGGYRRGSSPDSRTETMVTRRISRSSPDPNNGTQIQEDIDYNEVGEMDKDSTKREMRQFKDVPVKVSGSDAIPPTKQDGDGDDGRGLESISTFDSGYTSIVTAATLDDEEELLMKNNRPRKYQSTPQNSDKGIKKGVGRPKDTDKQSSILDYELNFKGSKKSQKILKASTNTGEPTRPQNGSQGKRITSWNILNSESGNRTESTNQTHQTSTSGQNHTMGPSRTTSEPRIKTQKTDGKEREDTEESTRFTERAITLLQNLGVIQSAAKLDLYQDKRVVCVANVLNNADTASKIDFLAGLMIGVSMDHDTKLNQIQNEILSLKTDLKKMDESHRRLIENQKEQLSLITSLISNLKIMTERGGKKDQPEPSGRTSMIKTKAKEEKIKKVRFDPLMETQGIEKNIPDLYRSIEKTPENDTQIKSEINRLNDESNATRLVPRRISSTMRSLIIIINNSNLSSKAKQSYINELKLCKSDEEVSELMDMFNEDVSSQ

SEQ ID NO: 49 - protein, 351 aa, Bovine parainfluenza virus 3
MSITNSTIYTFPESSFSENGNIEPLPLKVNEQRKAIPHIRVVKIGDPPKHGSRYLDVFLLGFFEMERSKDRYGSISDLDDDPSYKVCGSGSLPLGLARYTGNDQELLQAATKLDIEVRRTVKATEMIVYTVQNIKPELYPWSSRLRKGMLFDANKVALAPQCLPLDRGIKFRVIFVNCTAIGSITLFKIPKSMALLSLPNTISINLQVHIKTGVQTDSKGVVQILDEKGEKSLNFMVHLGLIKRKMGRMYSVEYCKQKIEKMRLLFSLGLVGGISFHVNATGSISKTLASQLAFKREICYPLMDLNPHLNSVIWASSVEITRVDAVLQPSLPGEFRYYPNIIAKGVGKIRQ

SEQ ID NO: 50 - protein, 540 aa, Bovine parainfluenza virus 3
MTITTTIIAILLIPPSFCQIDITKLQRVGVLVNNPKGMKISQNFETRYLILSLIPKIENSHSCGDQQINQYKKLLDRLIIPLYDGLKLQKDVIVVSHETHNNTNLRTKRFFGEIIGTIAIGIATSAQITAAVALVEAKQAKSDIEKLKEAIRDTNKAVQSIQSSVGNLIVAVKSVQDYVNNEIIPSITRLGCEAAGLQLGIALTQHYSELTNIFGDNIGTLKEKGIKLQGIASLYHTNITEIFTTSTVDQYDIYDLLFTESIKMRVIDVDLSDYSITLQVRLPLLTKLSNTQIYKVDSISYNIQGKEWYIPLPNHIMTKGAFLGGADIKECIEAFSSYICPSDPGYILNHEIENCLSGNITQCPKTVVTSDVVPRYAFVNGGLIANCITTTCTCNGIDNRINQSPDQGIKIITHKECQVIGINGMLFNTNREGTLATYTFDDIILNNSVALNPIDISMELNKAKLELEESKEWIKKSNQKLDSVGSWYQSSATITIIIVMIIILVIINITIIVVIIKFHRIQGKDQNDKNSEPYILTNRQ

SEQ ID NO: 51 - protein, 572 aa, Bovine parainfluenza virus 3
MEYWKHTNSINNTNNETETARGKHSSKVTNIIMYTFWTITLTILSVIFIMILTNLIQENNHNKLMLQEIRKEFAAIDTKIQRTSDDIGTSIQSGINTRLLTIQSHVQNYIPLSLTQQMSDLRKFINDLTNKREHQEVPIQRMTHDRGIEPLNPNKFWRCTSGNPSLTSSPKIRLIPGPGLLATSTTVNGCIRIPSLVINHLIYAYTSNLITQGCQDIGKSYQVLQIGIITINSDLVPDLNPRVTHTFNIDDNRRSCSLALLNTDVYQLCSTPKVDERSDYASTGIEDIVLDIVTNNGLIITTRFTNNNITFDKPYAALYPSVGPGIYYKDKVIFLGYGGLEHEENGDVICNTTGCPGKTQRDCNQASYSPWFSNRRMVNSIIVVDKGIDATFSLRVWTIPMSQNYWGSEGRLLLLGDRIYIYTRSTSWHSKLQLGVIDISDYTNIRINWTWHNVLSRPGNDECPWGHSCPDGCITGVYTDAYPLNPSGSVVSSVILDSQKSRENPIITYSTATNRINELAIYNRTLPAAYTTTNCITHYDKGYCFHIVEINHRSLNTFQPMLFKTEVPKNCS

SEQ ID NO: 52 - protein, 2233 aa, Bovine parainfluenza virus 3
MDTESHSGTTSDILYPECHLNSPIVKGKIAQLHTIMSLPQPYDMDDDSILIITRQKIKLNKLDKRQRSIRKLRSVLMERVSDLGKYTFIRYPEMSSEMFQLCIPGINNKINELLSKASKTYNQMTDGLRDLWVTILSKLASKNDGSNYDINEDISNISNVHMTYQSDKWYNPFKTWFTIKYDMRRLQKAKNEITFNRHKDYNLLEDQKNILLIHPELVLILDKQNYNGYIMTPELVLMYCDVVEGRWNISSCAKLDPKLQSMYYKGNNLWEIIDGLFSTLGERTFDIISLLEPLALSLIQTYDPVKQLRGAFLNHVLSEMELIFAAECTTEEIPNVDYIDKILDVFKESTIDEIAEIFSFFRTFGHPPLEASIAAEKVRKYMYTEKCLKFDTINKCHAIFCTIIINGYRERHGGQWPPVTLPVHAHEFIINAYGSNSAISYENAVDYYKSFIGIKFDKFIEPQLDEDLTIYMKDKALSPKKSNWDTVYPASNLLYRTNVSHDSRRLVEVFIADSKFDPHQVLDYVESGYWLDDPEFNISYSLKEKEIKQEGRLFAKMTYKMRATQVLSETLLANNIGKFFQENGMVKGEIELLKRLTTISMSGVPRYNEVYNNSKSHTEELQAYNAISSSNLSSNQKSKKFEFKSTDIYNDGYETVSCFLTTDLKKYCLNWRYESTALFGDTCNQIFGLKELFNWLHPRLEKSTIYVGDPYCPPSDIEHLPLDDHPDSGFYVHNPKGGIEGFCQKLWTLISISAIHLAAVKIGVRVTAMVQGDNQAIAVTTRVPNNYDYKVKKEIVYKDVVRFFDSLREVMDDLGHELKLNETIISSKMFIYSKRIYYDGRILPQALKALSRCVFWSETIIDETRSASSNLATSFAKAIENGYSPVLGYVCSIFKNIQQLYIALGMNINPTITQNIKDQYFRNIHWMQYASLIPASVGGFNYMAMSRCFVRNIGDPTVAALADIKRFIKANLLDRGVLYRIMNQEPGESSFLDWASDPYSCNLPQSQNITTMIKNITARNVLQDSPNPLLSGLFTSTMIEEDEELAEFLMDRRIILPRVAHDILDNSLTGIRNAIAGMLDTTKSLIRVGISRGGLTYNLLRKISNYDLVQYETLSKTLRLIVSDKIKYEDMCSVDLAISLRQKMWMHLSGGRMINGLETPDPLELLSGVIITGSEHCRICYSTEGESPYTWMYLPGNLNIGSAETGIASLRVPYFGSVTDERSEAQLGYIKNLSKPAKAAIRIAMIYTWAFGNDEISWMEASQIAQTRANFTLDSLKILTPVTTSTNLSHRLKDTATQMKFSSTSLIRVSRFITISNDNMSIKEANETKDTNLIYQQVMLTGLSVFEYLFRLEESTGHNPMVMHLHIEDGCCIKESYNDEHINPESTLELIKYPESNEFIYDKDPLKDIDLSKLMVIRDHSYTIDMNYWDDTDIVHAISICTAVTIADTMSQLDRDNLKELVVIANDDDINSLITEFLTLDILVFLKTFGGLLVNQFAYTLYGLKIEGRDPIWDYIMRTLKDTSHSVLKVLSNALSHPKVFKRFWDCGVLNPIYGPNTASQDQVKLALSICEYSLDLFMREWLNGASLEIYICDSDMEIANDRRQAFLSRHLAFVCCLAEIASFGPNLLNLTYLERLDELKQYLDLNIKEDPTLKYVQVSGLLIKSFPSTVTYVRKTAIKYLRIRGINPPETIEDWDPIEDENILDNIVKTVNDNCSDNQKRNKSSYFWGLALKNYQVVKIRSITSDSEVNEASNVTTHGMTLPQGGSYLSHQLRLFGVNSTSCLKALELSQILMREVKKDKDRLFLGEGAGAMLACYDATLGPAINYYNSGLNITDVIGQRELKIFPSEVSLVGKKLGNVTQILNRVRVLFNGNPNSTWIGNMECESLIWSELNDKSIGLVHCDMEGAIGKSEETVLHEHYSIIRITYLIGDDDVVLVSKIIPTITPNWSKILYLYKLYWKDVSVVSLKTSNPASTELYLISKDAYCTVMEPSNLVLSKLKRISSIEENNLLKWIILSKRKNNEWLQHEIKEGERDYGIMRPYHTALQIFGFQINLNHLAREFLSTPDLTNINNIIQSFTRTIKDVMFEWVNITHDNKRHKLGGRYNLFPLKNKGKLRLLSRRLVLSWISLSLSTRLLTGRFPDEKFENRAQTGYVSLADIDLESLKLLSRNIVKNYKEHIGLISYWFLTKEVKILMKLIGGVKLLGIPKQYKELEDRSSQGYEYDNEFDID

SEQ ID NO: 53 - protein, 47 aa, Bovine parainfluenza virus 3
ITIIIVMIIILVIINITIIVVIIKFHRIQGKDQNDKNSEPYILTNRQ

SEQ ID NO: 54 - DNA, 10 bp, Human parainfluenza virus 1
  source 1..10: mol_type = genomic DNA
agggttaaag

SEQ ID NO: 55 - DNA, 12 bp, Human parainfluenza virus 1
  source 1..12: mol_type = genomic DNA
aagtaagaaaaa

SEQ ID NO: 56 - DNA, 10 bp, Human parainfluenza virus 1
  source 1..10: mol_type = genomic DNA
agggtgaatg

SEQ ID NO: 57 - DNA, 12 bp, Human parainfluenza virus 1
  source 1..12: mol_type = genomic DNA
aattaagaaaaa

SEQ ID NO: 58 - DNA, 10 bp, Human parainfluenza virus 1
  source 1..10: mol_type = genomic DNA
agggtcaaag

SEQ ID NO: 59 - DNA, 12 bp, Human parainfluenza virus 1
  source 1..12: mol_type = genomic DNA
aaataagaaaaa

SEQ ID NO: 60 - DNA, 10 bp, Human parainfluenza virus 1
  source 1..10: mol_type = genomic DNA
agggacaaag

SEQ ID NO: 61 - DNA, 10 bp, Human parainfluenza virus 1
  source 1..10: mol_type = genomic DNA
agggttaaag

SEQ ID NO: 62 - DNA, 12 bp, Human parainfluenza virus 1
  source 1..12: mol_type = genomic DNA
gaataagaaaaa

SEQ ID NO: 63 - DNA, 10 bp, Human parainfluenza virus 1
  source 1..10: mol_type = genomic DNA
agggttaatg

SEQ ID NO: 64 - DNA, 12 bp, Human parainfluenza virus 1
  source 1..12: mol_type = genomic DNA
tagtaagaaaaa

SEQ ID NO: 65 - DNA, 14 bp, Human parainfluenza virus 2
  source 1..14: mol_type = genomic DNA
agattccggtgccg

SEQ ID NO: 66 - DNA, 14 bp, Human parainfluenza virus 2
  source 1..14: mol_type = genomic DNA
aatttaagaaaaaa

SEQ ID NO: 67 - DNA, 17 bp, Human parainfluenza virus 2
  source 1..17: mol_type = genomic DNA
aggcccggacgggttag

SEQ ID NO: 68 - DNA, 14 bp, Human parainfluenza virus 2
  source 1..14: mol_type = genomic DNA
aatttaataaaaaa

SEQ ID NO: 69 - DNA, 12 bp, Human parainfluenza virus 2
  source 1..12: mol_type = genomic DNA
aggtccgaaagc

SEQ ID NO: 70 - DNA, 15 bp, Human parainfluenza virus 2
  source 1..15: mol_type = genomic DNA
aatctaacaaaaaaa

SEQ ID NO: 71 - DNA, 12 bp, Human parainfluenza virus 2
  source 1..12: mol_type = genomic DNA
aggccaaattat

SEQ ID NO: 72 - DNA, 14 bp, Human parainfluenza virus 2
  source 1..14: mol_type = genomic DNA
aatttaagaaaaaa

SEQ ID NO: 73 - DNA, 12 bp, Human parainfluenza virus 2
  source 1..12: mol_type = genomic DNA
aagcacgaaccc

SEQ ID NO: 74 - DNA, 14 bp, Human parainfluenza virus 2
  source 1..14: mol_type = genomic DNA
tatttaagaaaaaa

SEQ ID NO: 75 - skipped

SEQ ID NO: 76 - DNA, 13 bp, Human parainfluenza virus 2
  source 1..13: mol_type = genomic DNA
tatttaagaaaaa

SEQ ID NO: 77 - DNA, 12 bp, Human parainfluenza virus 3
  source 1..12: mol_type = genomic DNA
aggattaaagac

SEQ ID NO: 78 - DNA, 12 bp, Human parainfluenza virus 3
  source 1..12: mol_type = genomic DNA
aaataagaaaaa

SEQ ID NO: 79 - DNA, 10 bp, Human parainfluenza virus 3
  source 1..10: mol_type = genomic DNA
aggattaaag

SEQ ID NO: 80 - DNA, 12 bp, Human parainfluenza virus 3
  source 1..12: mol_type = genomic DNA
aaataagaaaaa

SEQ ID NO: 81 - DNA, 10 bp, Human parainfluenza virus 3
  source 1..10: mol_type = genomic DNA
aggattaaag

SEQ ID NO: 82 - DNA, 20 bp, Human parainfluenza virus 3
  source 1..20: mol_type = genomic DNA
aaataaaggataatcaaaaa

SEQ ID NO: 83 - DNA, 10 bp, Human parainfluenza virus 3
  source 1..10: mol_type = genomic DNA
aggacaaaag

SEQ ID NO: 84 - DNA, 12 bp, Human parainfluenza virus 3
  source 1..12: mol_type = genomic DNA
aattataaaaaa

SEQ ID NO: 85 - DNA, 10 bp, Human parainfluenza virus 3
  source 1..10: mol_type = genomic DNA
aggagtaaag

SEQ ID NO: 86 - DNA, 12 bp, Human parainfluenza virus 3
  source 1..12: mol_type = genomic DNA
aaatataaaaaa

SEQ ID NO: 87 - DNA, 10 bp, Human parainfluenza virus 3
  source 1..10: mol_type = genomic DNA
aggagcaaag

SEQ ID NO: 88 - DNA, 13 bp, Human parainfluenza virus 3
  source 1..13: mol_type = genomic DNA
aaagtaagaaaaa

SEQ ID NO: 89 - DNA, 12 bp, Bovine parainfluenza virus 3
  source 1..12: mol_type = genomic DNA
aggattaaagaa

SEQ ID NO: 90 - DNA, 13 bp, Bovine parainfluenza virus 3
  source 1..13: mol_type = genomic DNA
caagtaagaaaaa

SEQ ID NO: 91 - DNA, 12 bp, Bovine parainfluenza virus 3
  source 1..12: mol_type = genomic DNA
aggattaatgga

SEQ ID NO: 92 - DNA, 13 bp, Bovine parainfluenza virus 3
  source 1..13: mol_type = genomic DNA
tgattaagaaaaa

SEQ ID NO: 93 - DNA, 12 bp, Bovine parainfluenza virus 3
  source 1..12: mol_type = genomic DNA
aggatgaaagga

SEQ ID NO: 94 - DNA, 13 bp, Bovine parainfluenza virus 3
  source 1..13: mol_type = genomic DNA
gaaaaatcaaaaa

SEQ ID NO: 95 - DNA, 12 bp, Bovine parainfluenza virus 3
  source 1..12: mol_type = genomic DNA
aggatcaaaggg

SEQ ID NO: 96 - DNA, 14 bp, Bovine parainfluenza virus 3
  source 1..14: mol_type = genomic DNA
aaaagtacaaaaaa

SEQ ID NO: 97 - DNA, 12 bp, Bovine parainfluenza virus 3
  source 1..12: mol_type = genomic DNA
aggaacaaagtt

SEQ ID NO: 98 - DNA, 14 bp, Bovine parainfluenza virus 3
  source 1..14: mol_type = genomic DNA
gaaataataaaaaa

SEQ ID NO: 99 - DNA, 12 bp, Bovine parainfluenza virus 3
  source 1..12: mol_type = genomic DNA
aggagaaaagtg

SEQ ID NO: 100 - DNA, 13 bp, Bovine parainfluenza virus 3
  source 1..13: mol_type = genomic DNA
aaagtaagaaaaa

SEQ ID NO: 101 - protein, 572 aa, Human parainfluenza virus 3
MEYWKHTNHGKDAGNELETSMATHGNKLTNKIIYILWTIILVLLSIVFIIVLINSIKSEKAHESLLQDINNEFMEITEKIQMASDNTNDLIQSGVNTRLLTIQSHVQNYIPISLTQQMSDLRKFISEITIRNDNQEVLPQRITHDVGIKPLNPDDFWRCTSGLPSLMKTPKIRLMPGPGLLAMPTTVDGCVRTPSLVINDLIYAYTSNLITRGCQDIGKSYQVLQIGIITVNSDLVPDLNPRISHTFNINDNRKSCSLALLNIDVYQLCSTPKVDERSDYASSGIEDIVLDIVNYDGSISTTRFKNNNISFDQPYAALYPSVGPGIYYKGKIIFLGYGGLEHPINENVICNTTGCPGKTQRDCNQASHSTWFSDRRMVNSIIVVDKGLNSIPKLKVWTISMRQNYWGSEGRLLLLGNKIYIYTRSTSWHSKLQLGIIDITDYSDIRIKWTWHNVLSRPGNNECPWGHSCPDGCITGVYTDAYPLNPTGSIVSSVILDSQKSRVNPVITYSTATERVNELAILNRTLSAGYTTTSCITHYNKGYCFHIVEINHKSLNTFQPMLFKTEIPKSCS

SEQ ID NO: 102 - protein, 1719 aa, Human parainfluenza virus 3
ATGGAATACTGGAAGCATACCAATCACGGAAAGGATGCTGGTAATGAGCTGGAGACGTCTATGGCTACTCATGGCAACAAGCTCACTAATAAGATAATATACATATTATGGACAATAATCCTGGTGTTATTATCAATAGTCTTCATCATAGTGCTAATTAATTCCATCAAAAGTGAAAAGGCCCACGAATCATTGCTGCAAGACATAAATAATGAGTTTATGGAAATTACAGAAAAGATCCAAATGGCATCGGATAATACCAATGATCTAATACAGTCAGGAGTGAATACAAGGCTTCTTACAATTCAGAGTCATGTCCAGAATTACATACCAATATCATTGACACAACAGATGTCAGATCTTAGGAAATTCATTAGTGAAATTACAATTAGAAATGATAATCAAGAAGTGCTGCCACAAAGAATAACACATGATGTAGGTATAAAACCTTTAAATCCAGATGATTTTTGGAGATGCACGTCTGGTCTTCCATCTTTAATGAAAACTCCAAAAATAAGGTTAATGCCAGGGCCGGGATTATTAGCTATGCCAACGACTGTTGATGGCTGTGTTAGAACTCCGTCTTTAGTTATAAATGATCTGATTTATGCTTATACCTCAAATCTAATTACTCGAGGTTGTCAGGATATAGGAAAATCATATCAAGTCTTACAGATAGGGATAATAACTGTAAACTCAGACTTGGTACCTGACTTAAATCCTAGGATCTCTCATACCTTTAACATAAATGACAATAGGAAGTCATGTTCTCTAGCACTCCTAAATATAGATGTATATCAACTGTGTTCAACTCCCAAAGTTGATGAAAGATCAGATTATGCATCATCAGGCATAGAAGATATTGTACTTGATATTGTCAATTATGATGGTTCAATCTCAACAACAAGATTTAAGAATAATAACATAAGCTTTGATCAACCATATGCTGCACTATACCCATCTGTTGGACCAGGGATATACTACAAAGGCAAAATAATATTTCTCGGGTATGGAGGTCTTGAACATCCAATAAATGAGAATGTAATCTGCAACACAACTGGGTGCCCCGGGAAAACACAGAGAGACTGTAATCAAGCATCTCATAGTACTTGGTTTTCAGATAGGAGGATGGTCAACTCCATCATTGTTGTTGACAAAGGCTTAAACTCAATTCCAAAATTGAAAGTATGGACGATATCTATGCGACAAAATTACTGGGGGTCAGAAGGAAGGTTACTTCTACTAGGTAACAAGATCTATATATATACAAGATCTACAAGTTGGCATAGCAAGTTACAATTAGGAATAATTGATATTACTGATTACAGTGATATAAGGATAAAATGGACATGGCATAATGTGCTATCAAGACCAGGAAACAATGAATGTCCATGGGGACATTCATGTCCAGATGGATGTATAACAGGAGTATATACTGATGCATATCCACTCAATCCCACAGGGAGCATTGTGTCATCTGTCATATTAGACTCACAAAAATCGAGAGTGAACCCAGTCATAACTTACTCAACAGCAACCGAAAGAGTAAACGAGCTGGCCATCCTAAACAGAACACTCTCAGCTGGATATACAACAACAAGCTGCATTACACACTATAACAAAGGATATTGTTTTCATATAGTAGAAATAAATCATAAAAGCTTAAACACATTTCAACCCATGTTGTTCAAAACAGAGATTCCAAAAAGCTGCAGTTAA

SEQ ID NO: 103 - protein, 65 aa, Sendai virus
VITIIVVMVVILVVIIVIIIVLYRLRRSMLMGNPDDRIPRDTYTLEPKIRHMYTNGGFDAMAEKR

SEQ ID NO: 104 - protein, 49 aa, Newcastle disease virus
IVLTIISLVFGILSLILACYLMYKQKAQQKTLLWLGNNTLDQMRATTKM

SEQ ID NO: 105 - protein, 594 aa, synthetic construct
  REGION 1..594: note = Recombinant RSV F
MELLILKANAITTILTAVTFCFASGQNITEEFYQSTCSAVSKGYLSALRTGWYTSVITIELSNIKENKCNGTDAKVKLIKQELDKYKNAVTELQLLMQSTPATNNRARRELPRFMNYTLNNAKKTNVTLSKKRKRRFLGFLLGVGSAIASGVAVSKVLHLEGEVNKIKSALLSTNKAVVSLSNGVSVLTSKVLDLKNYIDKQLLPIVNKQSCSISNIETVIEFQQKNNRLLEITREFSVNAGVTTPVSTYMLTNSELLSLINDMPITNDQKKLMSNNVQIVRQQSYSIMSIIKEEVLAYVVQLPLYGVIDTPCWKLHTSPLCTTNTKEGSNICLTRTDRGWYCDNAGSVSFFPQAETCKVQSNRVFCDTMNSLTLPSEVNLCNVDIFNPKYDCKIMTSKTDVSSSVITSLGAIVSCYGKTKCTASNKNRGIIKTFSNGCDYVSNKGVDTVSVGNTLYYVNKQEGKSLYVKGEPIINFYDPLVFPSDEFDASISQVNEKINQSLAFIRKSDELLHNVNAGKSTTNIMITTIIIVIIVILLSLIAVGLLLYCLYRLRRSMLMGNPDDRIPRDTYTLEPKIRHMYTNGGFDAMAEKR

SEQ ID NO: 106 - protein, 594 aa, synthetic construct
  REGION 1..594: note = Recombinant RSV F
MELLILKANAITTILTAVTFCFASGQNITEEFYQSTCSAVSKGYLSALRTGWYTSVITIELSNIKENKCNGTDAKVKLIKQELDKYKNAVTELQLLMQSTPATNNRARRELPRFMNYTLNNAKKTNVTLSKKRKRRFLGFLLGVGSAIASGVAVSKVLHLEGEVNKIKSALLSTNKAVVSLSNGVSVLTSKVLDLKNYIDKQLLPIVNKQSCSISNIETVIEFQQKNNRLLEITREFSVNAGVTTPVSTYMLTNSELLSLINDMPITNDQKKLMSNNVQIVRQQSYSIMSIIKEEVLAYVVQLPLYGVIDTPCWKLHTSPLCTTNTKEGSNICLTRTDRGWYCDNAGSVSFFPQAETCKVQSNRVFCDTMNSLTLPSEVNLCNVDIFNPKYDCKIMTSKTDVSSSVITSLGAIVSCYGKTKCTASNKNRGIIKTFSNGCDYVSNKGVDTVSVGNTLYYVNKQEGKSLYVKGEPIINFYDPLVFPSDEFDASISQVNEKINQSLAFIRKSDELLHNVNAGKSTTNIMITTVITIIVVMVVILVVIIVIIIVLYRLRRSMLMGNPDDRIPRDTYTLEPKIRHMYTNGGFDAMAEKR

SEQ ID NO: 107 - protein, 594 aa, synthetic construct
  REGION 1..594: note = Recombinant RSV F
MELLILKANAITTILTAVTFCFASGQNITEEFYQSTCSAVSKGYLSALRTGWYTSVITIELSNIKENKCNGTDAKVKLIKQELDKYKNAVTELQLLMQSTPATNNRARRELPRFMNYTLNNAKKTNVTLSKKRKRRFLGFLLGVGSAIASGVAVCKVLHLEGEVNKIKSALLSTNKAVVSLSNGVSVLTFKVLDLKNYIDKQLLPILNKQSCSISNIETVIEFQQKNNRLLEITREFSVNAGVTTPVSTYMLTNSELLSLINDMPITNDQKKLMSNNVQIVRQQSYSIMCIIKEEVLAYVVQLPLYGVIDTPCWKLHTSPLCTTNTKEGSNICLTRTDRGWYCDNAGSVSFFPQAETCKVQSNRVFCDTMNSLTLPSEVNLCNVDIFNPKYDCKIMTSKTDVSSSVITSLGAIVSCYGKTKCTASNKNRGIIKTFSNGCDYVSNKGVDTVSVGNTLYYVNKQEGKSLYVKGEPIINFYDPLVFPSDEFDASISQVNEKINQSLAFIRKSDELLHNVNAGKSTTNIMITTIIIVIIVILLSLIAVGLLLYCLYRLRRSMLMGNPDDRIPRDTYTLEPKIRHMYTNGGFDAMAEKR

SEQ ID NO: 108 - protein, 594 aa, synthetic construct
  REGION 1..594: note = Recombinant RSV F
MELLILKANAITTILTAVTFCFASGQNITEEFYQSTCSAVSKGYLSALRTGWYTSVITIELSNIKENKCNGTDAKVKLIKQELDKYKNAVTELQLLMQSTPATNNRARRELPRFMNYTLNNAKKTNVTLSKKRKRRFLGFLLGVGSAIASGVAVCKVLHLEGEVNKIKSALLSTNKAVVSLSNGVSVLTFKVLDLKNYIDKQLLPILNKQSCSISNIETVIEFQQKNNRLLEITREFSVNAGVTTPVSTYMLTNSELLSLINDMPITNDQKKLMSNNVQIVRQQSYSIMCIIKEEVLAYVVQLPLYGVIDTPCWKLHTSPLCTTNTKEGSNICLTRTDRGWYCDNAGSVSFFPQAETCKVQSNRVFCDTMNSLTLPSEVNLCNVDIFNPKYDCKIMTSKTDVSSSVITSLGAIVSCYGKTKCTASNKNRGIIKTFSNGCDYVSNKGVDTVSVGNTLYYVNKQEGKSLYVKGEPIINFYDPLVFPSDEFDASISQVNEKINQSLAFIRKSDELLHNVNAGKSTTNIMITTVITIIVVMVVILVVIIVIIIVLYRLRRSMLMGNPDDRIPRDTYTLEPKIRHMYTNGGFDAMAEKR

SEQ ID NO: 109 - protein, 578 aa, synthetic construct
  REGION 1..578: note = Recombinant RSV F
MELLILKANAITTILTAVTFCFASGQNITEEFYQSTCSAVSKGYLSALRTGWYTSVITIELSNIKENKCNGTDAKVKLIKQELDKYKNAVTELQLLMQSTPATNNRARRELPRFMNYTLNNAKKTNVTLSKKRKRRFLGFLLGVGSAIASGVAVSKVLHLEGEVNKIKSALLSTNKAVVSLSNGVSVLTSKVLDLKNYIDKQLLPIVNKQSCSISNIETVIEFQQKNNRLLEITREFSVNAGVTTPVSTYMLTNSELLSLINDMPITNDQKKLMSNNVQIVRQQSYSIMSIIKEEVLAYVVQLPLYGVIDTPCWKLHTSPLCTTNTKEGSNICLTRTDRGWYCDNAGSVSFFPQAETCKVQSNRVFCDTMNSLTLPSEVNLCNVDIFNPKYDCKIMTSKTDVSSSVITSLGAIVSCYGKTKCTASNKNRGIIKTFSNGCDYVSNKGVDTVSVGNTLYYVNKQEGKSLYVKGEPIINFYDPLVFPSDEFDASISQVNEKINQSLAFIRKSDELLHNVNAGKSTTNIMITTIIIVIIVILLSLIAVGLLLYCMYKQKAQQKTLLWLGNNTLDQMRATTKM

SEQ ID NO: 110 - protein, 578 aa, synthetic construct
  REGION 1..578: note = Recombinant RSV F
MELLILKANAITTILTAVTFCFASGQNITEEFYQSTCSAVSKGYLSALRTGWYTSVITIELSNIKENKCNGTDAKVKLIKQELDKYKNAVTELQLLMQSTPATNNRARRELPRFMNYTLNNAKKTNVTLSKKRKRRFLGFLLGVGSAIASGVAVSKVLHLEGEVNKIKSALLSTNKAVVSLSNGVSVLTSKVLDLKNYIDKQLLPIVNKQSCSISNIETVIEFQQKNNRLLEITREFSVNAGVTTPVSTYMLTNSELLSLINDMPITNDQKKLMSNNVQIVRQQSYSIMSIIKEEVLAYVVQLPLYGVIDTPCWKLHTSPLCTTNTKEGSNICLTRTDRGWYCDNAGSVSFFPQAETCKVQSNRVFCDTMNSLTLPSEVNLCNVDIFNPKYDCKIMTSKTDVSSSVITSLGAIVSCYGKTKCTASNKNRGIIKTFSNGCDYVSNKGVDTVSVGNTLYYVNKQEGKSLYVKGEPIINFYDPLVFPSDEFDASISQVNEKINQSLAFIRKSDELLHNVNAGKSTTNIMITTIVLTIISLVFGILSLILACYLMYKQKAQQKTLLWLGNNTLDQMRATTKM

SEQ ID NO: 111 - DNA, 49 bp, synthetic construct
  misc_feature 1..49: note = Oligonucleotide primer
  source 1..49: mol_type = other DNA
gcggccgccgtacgctatcagttggagaaggcgatattgttgatgccgg

SEQ ID NO: 112 - protein, 578 aa, synthetic construct
  REGION 1..578: note = Recombinant RSV F
MELLILKANAITTILTAVTFCFASGQNITEEFYQSTCSAVSKGYLSALRTGWYTSVITIELSNIKENKCNGTDAKVKLIKQELDKYKNAVTELQLLMQSTPATNNRARRELPRFMNYTLNNAKKTNVTLSKKRKRRFLGFLLGVGSAIASGVAVCKVLHLEGEVNKIKSALLSTNKAVVSLSNGVSVLTFKVLDLKNYIDKQLLPILNKQSCSISNIETVIEFQQKNNRLLEITREFSVNAGVTTPVSTYMLTNSELLSLINDMPITNDQKKLMSNNVQIVRQQSYSIMCIIKEEVLAYVVQLPLYGVIDTPCWKLHTSPLCTTNTKEGSNICLTRTDRGWYCDNAGSVSFFPQAETCKVQSNRVFCDTMNSLTLPSEVNLCNVDIFNPKYDCKIMTSKTDVSSSVITSLGAIVSCYGKTKCTASNKNRGIIKTFSNGCDYVSNKGVDTVSVGNTLYYVNKQEGKSLYVKGEPIINFYDPLVFPSDEFDASISQVNEKINQSLAFIRKSDELLHNVNAGKSTTNIMITTIIIVIIVILLSLIAVGLLLYCMYKQKAQQKTLLWLGNNTLDQMRATTKM

SEQ ID NO: 113 - protein, 594 aa, synthetic construct; identical to SEQ ID NO: 108
  REGION 1..594: note = Recombinant RSV F

SEQ ID NO: 114 - protein, 199 aa, Human parainfluenza virus 3
MLKTIKSWILGKRNQEINQLISPRPSTSLNSYSAPTPKKTYRKTTQSTQEPSNSVPPSVNQKSNQQKQVRKIVDQLTKIDSPGHHTNVQQKQKIEILIRKLYREDLGEEAAQIVELRLWSLEESPEASQILKMEPKTRRILISMKLERWIRTLLRGKCDNLQMFQARYQEVMTYLQQNKVETVIMEEAWNLSVHLIQDQ

SEQ ID NO: 115 - protein, 201 aa, Bovine parainfluenza virus 3
MFKTIKSWILGKRDQEINHLTSHRPSTSLNSYSAPTPKRTRQTAMKSTQEPQDLARQSTNLNPKQQKQARKIVDQLTKIDSLGHHTNVPQRQKIEMLIRRLYREDIGEEAAQIVELRLWSLEESPEAAQILTMEPKSRKILITMKLERWIRTLLRGKCDNLKMFQSRYQEVMPFLQQNKMETVMMEEAWNLSVHLIQDIPV

SEQ ID NO: 116 - protein, 412 aa, Bovine parainfluenza virus 3
MEDNVQNNQIMDSWEEGSGDKSSDISSALDIIEFILSTDSQENTADSNEINTGTTRLSTTIYQPESKTTETSKENSGPANKNRQFGASHERATETKDRNVNQETVQGGYRRGSSPDSRTETMVTRRISRSSPDPNNGTQIQEDIDYNEVGEMDKDSTKREMRQFKDVPVKVSGSDAIPPTKQDGDGDDGRGLESISTFDSGYTSIVTAATLDDEEELLMKNNRPRKYQSTPQNSDKGIKKGGWKAKRHRQTIINIGLRTQLQRIEEEPENPQSQHEYRRTNKTTEWIPGEENHILEHPQQRERQSNRINKPNPSDINLGTEPHNGTKQNNLRTKDQDTKDGWKGKRGHRREHSIYRKGDYIITESWCNPICSKIRPIPRQESCVCGECPKQCRYCIKDRLPSRFDDRSVNGS

SEQ ID NO: 117 - DNA, 46 bp, human parainfluenza virus 2
  source 1..46: mol_type = genomic DNA
ttaaaagaagttaagtaaaatttaaagaacacaatagagaaaacct

SEQ ID NO: 118 - DNA, 28 bp, human parainfluenza virus 2
  source 1..28: mol_type = genomic DNA
ctaaacattcaataataaatcaaagttc

SEQ ID NO: 119 - skipped

SEQ ID NO: 120 - DNA, 42 bp, human parainfluenza virus 2
  source 1..42: mol_type = genomic DNA
taatctttatataatgtaacaatactactaagattataatat

SEQ ID NO: 121 - DNA, 34 bp, synthetic construct
  misc_feature 1..34: note = Oligonucleotide primer
  source 1..34: mol_type = other DNA
aagaagaccaagttgagccagaagaggtacgaag

SEQ ID NO: 122 - DNA, 34 bp, synthetic construct
  misc_feature 1..34: note = Oligonucleotide primer
  source 1..34: mol_type = other DNA
cttcgtacctcttctggctcaacttggtcttctt

SEQ ID NO: 123 - DNA, 51 bp, synthetic construct
  misc_feature 1..51: note = Oligonucleotide primer
  source 1..51: mol_type = other DNA
ccagctaacataggagggttcaacgcgatgtctacagctagatgttttgtc

SEQ ID NO: 124 - DNA, 51 bp, synthetic construct
  misc_feature 1..51: note = Oligonucleotide primer
  source 1..51: mol_type = other DNA
gacaaaacatctagctgtagacatcgcgttgaaccctcctatgttagctgg

SEQ ID NO: 125 - DNA, 12 bp, Human parainfluenza virus 1
  source 1..12: mol_type = genomic DNA
aagtaagaaaaa

SEQ ID NO: 126 - DNA, 10 bp, Human parainfluenza virus 1
  source 1..10: mol_type = genomic DNA
agggtgaatg

SEQ ID NO: 127 - DNA, 46 bp, synthetic construct
  misc_feature 1..46: note = Oligonucleotide primer
  source 1..46: mol_type = other DNA
acgcgtcccgggaacaatggaactgctgatcctgaaggccaacgcc

SEQ ID NO: 128 - DNA, 73 bp, synthetic construct
  misc_feature 1..73: note = Oligonucleotide primer
  source 1..73: mol_type = other DNA
acgcgtcgtacgcattcaccctaagtttttcttactttctatcagttggagaaggcgatattgttgatgccgg

SEQ ID NO: 129 - DNA, 48 bp, synthetic construct
  misc_feature 1..48: note = Oligonucleotide primer
  source 1..48: mol_type = other DNA
ggcgcgcccccgggaacaatggaactgctgatcctgaaggccaacgcc

SEQ ID NO: 130 - DNA, 79 bp, synthetic construct
  misc_feature 1..79: note = Oligonucleotide primer
  source 1..79: mol_type = other DNA
ggcgcgcccgtacgccattcaccctaagtttttcttacttgattctatcagttggagaaggcgatattgttgatgccgg

SEQ ID NO: 131 - DNA, 72 bp, synthetic construct
  misc_feature 1..72: note = Oligonucleotide primer
  source 1..72: mol_type = other DNA
gcggccgcccgggaagtaagaaaaacttagggtgaatgaacaatggaactgctgatcctgaaggccaacgcc

SEQ ID NO: 132 - protein, 31 aa, synthetic construct
  REGION 1..31: note = linker and foldon domain
SAIGGYIPEAPRDGQAYVRKDGEWVLLSTFL

SEQ ID NO: 133 - protein, 586 aa, synthetic construct
  REGION 1..586: note = Recombinant RSV F
MELLILKANAITTILTAVTFCFASGQNITEEFYQSTCSAVSKGYLSALRTGWYTSVITIELSNIKENKCNGTDAKVKLIKQELDKYKNAVTELQLLMQSTPATNNRARRELPRFMNYTLNNAKKTNVTLSKKRKRRFLGFLLGVGSAIASGVAVCKVLHLEGEVNKIKSALLSTNKAVVSLSNGVSVLTFKVLDLKNYIDKQLLPILNKQSCSISNIETVIEFQQKNNRLLEITREFSVNAGVTTPVSTYMLTNSELLSLINDMPITNDQKKLMSNNVQIVRQQSYSIMCIIKEEVLAYVVQLPLYGVIDTPCWKLHTSPLCTTNTKEGSNICLTRTDRGWYCDNAGSVSFFPQAETCKVQSNRVFCDTMNSLTLPSEVNLCNVDIFNPKYDCKIMTSKTDVSSSVITSLGAIVSCYGKTKCTASNKNRGIIKTFSNGCDYVSNKGVDTVSVGNTLYYVNKQEGKSLYVKGEPIINFYDPLVFPSDEFDASISQVNEKINQSLAFIRKSDELLHNVNAGKSTTNIMITTIIIVIIVILLSLIAVGLLLYCRVRRLLVMINSTHNSPVNAYTLESRMRNPYMGNNSN

SEQ ID NO: 134 - DNA, 1764 bp, synthetic construct
  misc_feature 1..1764: note = recombinant RSV F
  source 1..1764: mol_type = other DNA
atggaactgctgatcctgaaagccaacgctattactactatcctgaccgccgtgacattttgcttcgcatctggacagaacattactgaggaattctaccagtcaacatgcagcgccgtgtccaaaggatacctgagcgccctgcggaccggctggtatacatcagtgattactatcgagctgtccaacatcaaggaaaacaaatgtaatgggaccgacgcaaaggtgaaactgatcaagcaggagctggataagtacaaaaatgccgtgacagaactgcagctgctgatgcagtccacaccagcaactaacaatcgcgcccggagagagctgccccggttcatgaactataccctgaacaatgctaagaaaaccaatgtgacactgtccaagaaacgcaagaggcgcttcctgggatttctgctgggcgtggggtctgccatcgctagtggagtggccgtctgcaaagtcctgcacctggagggcgaagtgaacaagatcaaaagcgccctgctgtccactaacaaggcagtggtcagtctgtcaaatggcgtgtccgtcctgaccttcaaggtgctggacctgaaaaattatattgataagcagctgctgcctatcctgaacaaacagagctgctccatttctaatatcgagacagtgatcgaattccagcagaagaacaatagactgctggagattaccagagagttcagcgtgaacgccggcgtcaccacacccgtgtccacctacatgctgacaaatagtgagctgctgtcactgattaacgacatgcctatcaccaatgatcagaagaaactgatgtccaacaatgtgcagatcgtcagacagcagagttactcaatcatgtgcatcattaaggaggaagtcctggcctacgtggtccagctgccactgtatggcgtgatcgacaccccctgctggaaactgcatacatctcctctgtgcactaccaacacaaaggaaggaagtaatatctgcctgactcgaaccgaccggggatggtactgtgataacgcaggcagcgtgtccttctttccacaggccgagacctgcaaggtccagagcaacagggtgttctgtgacactatgaatagcctgaccctgccttccgaagtcaacctgtgcaatgtggacatctttaatccaaagtacgattgtaagatcatgactagcaagaccgatgtcagctcctctgtgattacttctctgggggccatcgtgagttgctacggaaagacaaaatgtactgccagcaacaaaaatcgcggcatcattaagaccttctccaacgggtgcgactatgtctctaacaagggcgtggatacagtgagtgtcgggaacactctgtactatgtcaataagcaggagggaaaaagcctgtacgtgaagggcgaacccatcattaacttctatgaccccctggtgttcccttccgacgagtttgatgcatctattagtcaggtgaacgaaaaaatcaatcagagtctggcctttattcggaagtcagatgagctgctgcacaacgtgaatgctggcaaatctacaactaacatcatgatcaccacaatcatcatcgtgattatcgtcattctgctgtcactgatcgctgtggggctgctgctgtactgtcgagtgcggagactgctggtcatgattaacagcacccacaattcccccgtcaacgcctacacactggagtctaggatgcgcaatccttatatggggaacaatagcaactgatag

SEQ ID NO: 135 - protein, 588 aa, synthetic construct
  REGION 1..588: note = recombinant RSV F
MELLILKANAITTILTAVTFCFASGQNITEEFYQSTCSAVSKGYLSALRTGWYTSVITIELSNIKENKCNGTDAKVKLIKQELDKYKNAVTELQLLMQSTPATNNRARRELPRFMNYTLNNAKKTNVTLSKKRKRRFLGFLLGVGSAIASGVAVCKVLHLEGEVNKIKSALLSTNKAVVSLSNGVSVLTFKVLDLKNYIDKQLLPILNKQSCSISNIETVIEFQQKNNRLLEITREFSVNAGVTTPVSTYMLTNSELLSLINDMPITNDQKKLMSNNVQIVRQQSYSIMCIIKEEVLAYVVQLPLYGVIDTPCWKLHTSPLCTTNTKEGSNICLTRTDRGWYCDNAGSVSFFPQAETCKVQSNRVFCDTMNSLTLPSEVNLCNVDIFNPKYDCKIMTSKTDVSSSVITSLGAIVSCYGKTKCTASNKNRGIIKTFSNGCDYVSNKGVDTVSVGNTLYYVNKQEGKSLYVKGEPIINFYDPLVFPSDEFDASISQVNEKINQSLAFIRKSDELLHNVNAGKSTTNIMITTQIIMIIIVCILIIIICGILYYLYRVRRLLVMINSTHNSPVNAYTLESRMRNPYMGNNSN

SEQ ID NO: 136 - DNA, 1770 bp, synthetic construct
  misc_feature 1..1770: note = recombinant RSV F
  source 1..1770: mol_type = other DNA
atggaactgctgatcctgaaagccaacgctattactactatcctgaccgccgtgacattttgcttcgcatctggacagaacattactgaggaattctaccagtcaacatgcagcgccgtgtccaaaggatacctgagcgccctgcggaccggctggtatacatcagtgattactatcgagctgtccaacatcaaggaaaacaaatgtaatgggaccgacgcaaaggtgaaactgatcaagcaggagctggataagtacaaaaatgccgtgacagaactgcagctgctgatgcagtccacaccagcaactaacaatcgcgcccggagagagctgccccggttcatgaactataccctgaacaatgctaagaaaaccaatgtgacactgtccaagaaacgcaagaggcgcttcctgggatttctgctgggcgtggggtctgccatcgctagtggagtggccgtctgcaaagtcctgcacctggagggcgaagtgaacaagatcaaaagcgccctgctgtccactaacaaggcagtggtcagtctgtcaaatggcgtgtccgtcctgaccttcaaggtgctggacctgaaaaattatattgataagcagctgctgcctatcctgaacaaacagagctgctccatttctaatatcgagacagtgatcgaattccagcagaagaacaatagactgctggagattaccagagagttcagcgtgaacgccggcgtcaccacacccgtgtccacctacatgctgacaaatagtgagctgctgtcactgattaacgacatgcctatcaccaatgatcagaagaaactgatgtccaacaatgtgcagatcgtcagacagcagagttactcaatcatgtgcatcattaaggaggaagtcctggcctacgtggtccagctgccactgtatggcgtgatcgacaccccctgctggaaactgcatacatctcctctgtgcactaccaacacaaaggaaggaagtaatatctgcctgactcgaaccgaccggggatggtactgtgataacgcaggcagcgtgtccttctttccacaggccgagacctgcaaggtccagagcaacagggtgttctgtgacactatgaatagcctgaccctgccttccgaagtcaacctgtgcaatgtggacatctttaatccaaagtacgattgtaagatcatgactagcaagaccgatgtcagctcctctgtgattacttctctgggggccatcgtgagttgctacggaaagacaaaatgtactgccagcaacaaaaatcgcggcatcattaagaccttctccaacgggtgcgactatgtctctaacaagggcgtggatacagtgagtgtcgggaacactctgtactatgtcaataagcaggagggaaaaagcctgtacgtgaagggcgaacccatcattaacttctatgaccccctggtgttcccttccgacgagtttgatgcatctattagtcaggtgaacgaaaaaatcaatcagagtctggcctttattcggaagtcagatgagctgctgcacaacgtgaatgctggcaaatctacaactaacatcatgatcaccacacagatcattatgatcattatcgtgtgcattctgattatcattatctgtggcatcctgtactatctgtaccgagtgcggagactgctggtcatgattaacagcacccacaattcccccgtcaacgcctacacactggagtctaggatgcgcaatccttatatggggaacaatagcaactgatag

SEQ ID NO: 137 - DNA, 1731 bp, synthetic construct
  misc_feature 1..1731: note = recombinant RSV F
  source 1..1731: mol_type = other DNA
atggaactgctgatcctgaaagccaacgctattactactatcctgaccgccgtgacattttgcttcgcatctggacagaacattactgaggaattctaccagtcaacatgcagcgccgtgtccaaaggatacctgagcgccctgcggaccggctggtatacatcagtgattactatcgagctgtccaacatcaaggaaaacaaatgtaatgggaccgacgcaaaggtgaaactgatcaagcaggagctggataagtacaaaaatgccgtgacagaactgcagctgctgatgcagtccacaccagcaactaacaatcgcgcccggagagagctgccccggttcatgaactataccctgaacaatgctaagaaaaccaatgtgacactgtccaagaaacgcaagaggcgcttcctgggatttctgctgggcgtggggtctgccatcgctagtggagtggccgtctgcaaagtcctgcacctggagggcgaagtgaacaagatcaaaagcgccctgctgtccactaacaaggcagtggtcagtctgtcaaatggcgtgtccgtcctgacctccaaggtgctggacctgaaaaattatattgataagcagctgctgcctatcgtcaacaaacagagctgctccatttctaatatcgagacagtgatcgaattccagcagaagaacaatagactgctggagattaccagagagttcagcgtgaacgccggcgtcaccacacccgtgtccacctacatgctgacaaatagtgagctgctgtcactgattaacgacatgcctatcaccaatgatcagaagaaactgatgtccaacaatgtgcagatcgtcagacagcagagttactcaatcatgtgcatcattaaggaggaagtcctggcctacgtggtccagctgccactgtatggcgtgatcgacaccccctgctggaaactgcatacatctcctctgtgcactaccaacacaaaggaaggaagtaatatctgcctgactcgaaccgaccggggatggtactgtgataacgcaggcagcgtgtccttctttccacaggccgagacctgcaaggtccagagcaacagggtgttctgtgacactatgaatagcctgaccctgccttccgaagtcaacctgtgcaatgtggacatctttaatccaaagtacgattgtaagatcatgactagcaagaccgatgtcagctcctctgtgattacttctctgggggccatcgtgagttgctacggaaagacaaaatgtactgccagcaacaaaaatcgcggcatcattaagaccttctccaacgggtgcgactatgtctctaacaagggcgtggatacagtgagtgtcgggaacactctgtactatgtcaataagcaggagggaaaaagcctgtacgtgaagggcgaacccatcattaacttctatgaccccctggtgttcccttccgacgagtttgatgcatctattagtcaggtgaacgaaaaaatcaatcagagtctggcctttattcggaagtcagatgagctgctgcacaacgtgaatgctggcaaatctacaactaacatcatgatcaccacaatcaccatcattatcgtgatgattatcattctggtcatcattaacatcacaatcattgtggtcatcattaagttccaccggattcagggcaaggaccagaacgataaaaatagcgagccctacatcctgaccaatagacagtga

SEQ ID NO: 138 - DNA, 15 bp, Human parainfluenza virus 1
  source 1..15: mol_type = genomic DNA
agggttaaagtaata

SEQ ID NO: 139 - DNA, 21 bp, Human parainfluenza virus 1
  source 1..21: mol_type = genomic DNA
taaatacgcgtcccgggaaca

SEQ ID NO: 140 - DNA, 38 bp, Human parainfluenza virus 1
  source 1..38: mol_type = genomic DNA
aaagtaagaaaaacttagggtgaatgcgtacgacgcgt

SEQ ID NO: 141 - DNA, 14 bp, Human parainfluenza virus 1
  source 1..14: mol_type = genomic DNA
agggtgaatgacaa

SEQ ID NO: 142 - DNA, 21 bp, Human parainfluenza virus 1
  source 1..21: mol_type = genomic DNA
cagggcgcgcccccgggaaca

SEQ ID NO: 143 - DNA, 44 bp, Human parainfluenza virus 1
  source 1..44: mol_type = genomic DNA
aatcaagtaagaaaaacttagggtgaatggcgtacgggcgcgcc

SEQ ID NO: 144 - DNA, 42 bp, Human parainfluenza virus 1
  source 1..42: mol_type = genomic DNA
gcggccgcccgggaagtaagaaaaacttagggtgaatgaaca

SEQ ID NO: 145 - DNA, 31 bp, Human parainfluenza virus 1
  source 1..31: mol_type = genomic DNA
cgtacggcggccgcaaaacaattaagaaaaa

SEQ ID NO: 146 - DNA, 15 bp, Human parainfluenza virus 1
  source 1..15: mol_type = genomic DNA
acgcgtgccgccacc

SEQ ID NO: 147 - DNA, 37 bp, Human parainfluenza virus 1
  source 1..37: mol_type = genomic DNA
aaaagtaagaaaaacttagggtgaatgacgcgtaatg

SEQ ID NO: 148 - DNA, 64 bp, Human parainfluenza virus 3
  source 1..64: mol_type = genomic DNA
cttaggattaaagacattgactagaaggtcaagaaaagggaactctataatttcaaaaatgttg

SEQ ID NO: 149 - DNA, 20 bp, Human parainfluenza virus 3
  source 1..20: mol_type = genomic DNA
gcttagcgccgccaccatgg

SEQ ID NO: 150 - DNA, 49 bp, Human parainfluenza virus 3
  source 1..49: mol_type = genomic DNA
tgatagataataaataagaaaaacttaggattaaagaagcttagcaatg

SEQ ID NO: 151 - protein, 63 aa, Bovine parainfluenza virus 3
NQKLDSVGSWYQSSATITIIIVMIIILVIINITIIVVIIKFHRIQGKDQNDKNSEPYILTNRQ

SEQ ID NO: 152 - protein, 79 aa, Human parainfluenza virus 1
LMKARAIISAVGGWHNTESTQIIMIIIVCILIIIICGILYYLYRVRRLLVMINSTHNSPVNAYTLESRMRNPYMGNNSN

SEQ ID NO: 153 - protein, 66 aa, Human parainfluenza virus 3
IRRSNQKLDSIGNWHQSSTTIIIILIMIIILFIINITIITIAIKYYRIQKRNRVDQNDKPYVLTNK